European Patent Application EP 4 219 546 A2, published August 2, 2023. Title: Production Cell Line Enhancers. Applicant: Regeneron Pharmaceuticals, Inc. Application EP. The sequence listing filed with the application follows.

SEQUENCE LISTING (46 sequences)

SEQ ID NO: 1 - protein, 577 aa, Mus musculus
MPFRLLIPLGLVCVLLPLHHGAPGPDGTAPDPAHYRERVKAMFYHAYDSYLENAFPYDELRPLTCDGHDTWGSFSLTLIDALDTLLILGNTSEFQRVVEVLQDNVDFDIDVNASVFETNIRVVGGLLSAHLLSKKAGVEVEAGWPCSGPLLRMAEEAARKLLPAFQTPTGMPYGTVNLLHGVNPGETPVTCTAGIGTFIVEFATLSSLTGDPVFEDVARVALMRLWESRSDIGLVGNHIDVLTGKWVAQDAGIGAGVDSYFEYLVKGAILLQDKKLMAMFLEYNKAIRNYTHFDDWYLWVQMYKGTVSMPVFQSLEAYWPGLQSLIGDIDNAMRTFLNYYTVWKQFGGLPEFYNIPQGYTVEKREGYPLRPELIESAMYLYRATGDPTLLELGRDAVESIEKISKVECGFATIKDLRDHKLDNRMESFFLAETVKYLYLLFHPNNFIHNNGSTFDSVMTPHGECILGAGGYIFNTEAHPIDPAALHCCRRLKEEQWEVEDLIKEFYSLKQSRPKRAQRKTVRSGPWEPQSGPATLSSPANQPREKQPAQQRTPLLSCPSQPFTSKLALLGQVFLDSS

SEQ ID NO: 2 - protein, 576 aa, Rattus norvegicus
MPFRLLIPLGLVCVLLPLHHGAPGPEGTAPDPAHYRERVKAMFYHAYDSYLENAFPYDELRPLTCDGHDTWGSFSLTLIDALDTLLILGNTSEFQRVVEVLQDNVDFDIDVNASVFETNIRVVGGLLSAHLLSKKAGVEVEAGWPCSGPLLRMAEEAARKLLPAFQTPTGMPYGTVNLLHGVNPGETPVTCTAGIGTFIVEFATLSSLTGDPVFEDVARVALMRLWESRSDIGLVGNHIDVLTGKWVAQDAGIGAGVDSYFEYLVKGAILLQDKKLMAMFLEYNKAIRNYTHFDDWYLWVQMYKGTVSMPVFQSLEAYWPGLQSLIGDIDNAMRTFLNYYTVWKQFGGLPEFYNIPQGYTVEKREGYPLRPELIESAMYLYRATGDPTLLELGRDAVESIEKISKVECGFATIKDLRDHKLDNRMESFFLAETVKYLYLLFHPNNFIHNNGSTFDSVMTPHGECILGAGGYIFNTEAHPIDPAALHCCRRLKEEQWEVEDLIKEFYSLRQSRSRAQRKTVSSGPWEPPAGPGTLSSPENQPREKQPARQRAPLLSCPSQPFTSKLALLGQVFLDSS

SEQ ID NO: 3 - protein, 578 aa, Cricetulus griseus
MPFRLLIPLGLVCVFLPLHHGAPGPDGTAPDPAHYRERVKAMFYHAYDSYLENAFPYDELRPLTCDGHDTWGSFSLTLIDALDTLLILGNTSEFQRVVEVLQDNVDFDIDVNASVFETNIRVVGGLLSAHLLSKKAGVEVEAGWPCSGPLLRMAEEAARKLLPAFQTPTGMPYGTVNLLHGVNPGETPVTCTAGIGTFIVEFATLSSLTGDPVFEDVARLALMRLWESRSDIGLVGNHIDVLTGKWVAQDAGIGAGVDSYFEYLVKGAILLQDKKLMAMFLEYNRAIRNYTHFDDWYLWVQMYKGTVSMPVFQSLEAYWPGLQSLIGDIDNAMRTFLNYYTVWKQFGGLPEFYNIAQGYTVEKREGYPLRPELIESAMYLYRATGDPTLLELGRDAVESIEKISKVECGFATIKDLRDHKLDNRMESFFLAETVKYLYLLFHPNNFIHNNGSTFDSVMTPHGECILGAGGYIFNTEAHPIDPAALHCCRRLKEEQWEVEDLMRELHSLKQSRSRAQRKTTSSGPWEPPAGPGSPSAPGKQDQPREKQPAKQRTPLLSCPSQPFTSKLALLGQVFLDSS

SEQ ID NO: 4 - protein, 578 aa, Homo sapiens [sequence omitted]

SEQ ID NO: 5 - protein, 578 aa, Pan troglodytes
MPFRLLIPLGLLCALLPLHHGAPGPDGSAPDPAHYRERVKAMFYHAYDSYLENAFPFDELRPLTCDGHDTWGSFSLTLIDALDTLLILGNVSEFQRVVEVLQDSVDFDIDVNASVFETNIRVVGGLLSAHLLSKKAGVEVEAGWPCSGPLLRMAEEAARKLLPAFQTPTGMPYGTVNLLHGVNPGETPVTCTAGIGTFIVEFATLSSLTGDPVFEDVARVALMRLWESRSDIGLVGNHIDVLTGKWVAQDAGIGAGVDSYFEYLVKGAILLQDKKLMAMFLEYNKAIRNYTRFDDWYLWVQMYKGTVSMPVFQSLEAYWPGLQSLIGDIDNAMRTFLNYYTVWKQFGGLPEFYNIPQGYTVEKREGYPLRPELIESAMYLYRATGDPTLLELGRDAVESIEKISKVECGFATIKDLRDHKLDNRMESFFLAETVKYLYLLFDPTNFIHNNGSTFDAVITPYGECILGAGGYIFNTEAHPIDPAALHCCQRLKEEQWEVEDLMREFYSLKRSRSKFQKKTVSSGPWEPPARPGTLFSPENHDQARERKPAKQKVPLLSCPSQPFTSKLALLGQVFLDSS

SEQ ID NO: 6 - protein, 513 aa, Pongo pygmaeus
MNTLSCSLFSLTLIDALDTLLILGNVSEFQRVVEVLQDNVDFDIDVNASVFETNIRVVGGLLSAHLLSKKAGVEVEAGWPCSGPLLRMAEEAARKLLPAFQTPTGMPYGTVNLLHGVNPGETPVTCTAGIGTFIVEFATLSSLTGDPVFEDVARVALMRLWESRSDIGLVGNHIDVLTGKWVAQDAGIGAGVDSYFEYLVKGAILLQDKKLMAMFLEYNKAIRNYTRFDDWYLWVQMYKGTVSMPVFQSLEAYWPGLQSLIGDIDNAMRTFLNYYTVWKQFGGLPEFYNIPQGYTVEKREGYPLRPELIESAMYLYRATGDPTLLELGRDAVESIEKISKVECGFATIKDLRDHKLDNRMESFFLAETVKYLYLLFDPTNFIHNNGSTFDAVITPYGECILGAGGYIFNTEAHPIDPAALHCCQRLKEEQWEVEDLMREFYSLKRNRSKFQKKTVSSGPWEPPARPGTLFSPENHDQARGRKPAKQKVPLLSCPSQPFTSKLALLGQVFLDSS

SEQ ID NO: 7 - protein, 572 aa, Danio rerio
LYYLPLFTSRYFMLTFLFSAIFCAAYLSPIISHVKGRDFTEQEMSHYRDRVKSMFYHAYNSYLDNAYPYDELRPLTCDGQDTWGSFSLTLIDALDTLLILGNHTEFQRVATLLQDTVDFDIDVNASVFETNIRVVGGLLSAHLLSKRAGMKVEEGWPCSGPLLRMAEDAARKLLPAFQTPTGMPYGTVNLLRGVNPGETPVTCTAGVGTFILEFSTLSRLTGDPVFENVARKALRALWRTRSDIGLVGNHIDVITSKWVAQDAGIGAGVDSYFEYLVRGAIMLQDEELLTMFYEFDKSIKNYTKFDDWYLWVQMHKGTVSMPVFQSLEAFWPGMQSLIGDISSATKSFHNYYSVWRQFGGLPEFYSIPQGYTVDKREGYPLRPELIESAMYLYKATGDPSFIQLGRDAVESIDRISRVNCGFATVKDVRDHKLDNRMESFFLAETIKYLYLLFDPDNFLHNTGTEFELGGLRGDCILSAGGYVFNTEAHPLDPAALHCCSREQQDRREIQDILLSFSQPHTEEPSRDQSAGGSPESIALKPGEQRKAPVLSCPTQPFSAKLAVMGQVFSDNS

SEQ ID NO: 8 - protein, 579 aa, synthetic construct
  REGION 1..579: note = Consensus sequence
  SITE 12: note = MISC_FEATURE - V or L
  SITE 14: note = MISC_FEATURE - V or A
  SITE 15: note = MISC_FEATURE - L or F
  SITE 26: note = MISC_FEATURE - D or E
  SITE 28: note = MISC_FEATURE - T or S
  SITE 57: note = MISC_FEATURE - Y or F
  SITE 91: note = MISC_FEATURE - T or V
  SITE 104: note = MISC_FEATURE - N or S
  SITE 220: note = MISC_FEATURE - V or L
  SITE 285: note = MISC_FEATURE - K or R
  SITE 292: note = MISC_FEATURE - H or R
  SITE 356: note = MISC_FEATURE - P or A
  SITE 442: note = MISC_FEATURE - H or D
  SITE 444: note = MISC_FEATURE - N or T
  SITE 456: note = MISC_FEATURE - S, T, or A
  SITE 458: note = MISC_FEATURE - M or I
  SITE 461: note = MISC_FEATURE - H or Y
  SITE 489: note = MISC_FEATURE - R or Q
  SITE 502: note = MISC_FEATURE - I or M
  SITE 503: note = MISC_FEATURE - K or R
  SITE 505: note = MISC_FEATURE - F or L
  SITE 506: note = MISC_FEATURE - Y or H
  SITE 509: note = MISC_FEATURE - K or R
  SITE 510: note = MISC_FEATURE - Q or R
  SITE 513: note = MISC_FEATURE - P or S
  REGION 514..516: note = MISC_FEATURE - KRA, RA, or KF (one amino acid may be missing)
  SITE 518: note = MISC_FEATURE - R or K
  SITE 519: note = MISC_FEATURE - K or N
  SITE 522: note = MISC_FEATURE - R or S
  SITE 529: note = MISC_FEATURE - Q or P
  SITE 530: note = MISC_FEATURE - S or A
  SITE 531: note = MISC_FEATURE - G or R
  SITE 533: note = MISC_FEATURE - A or G
  SITE 534: note = MISC_FEATURE - T or S
  SITE 535: note = MISC_FEATURE - L or P
  SITE 536: note = MISC_FEATURE - S or F
  SITE 537: note = MISC_FEATURE - S or A
  REGION 539..542: note = MISC_FEATURE - AN, EN, GKQD, or ENHD (two amino acids may be missing)
  SITE 544: note = MISC_FEATURE - P or A
  SITE 547: note = MISC_FEATURE - K or R
  SITE 548: note = MISC_FEATURE - Q or K
  SITE 551: note = MISC_FEATURE - Q, R, or K
  SITE 553: note = MISC_FEATURE - R or K
  SITE 554: note = MISC_FEATURE - T, A, or V
MPFRLLIPLGLXCXXLPLHHGAPGPXGXAPDPAHYRERVKAMFYHAYDSYLENAFPXDELRPLTCDGHDTWGSFSLTLIDALDTLLILGNXSEFQRVVEVLQDXVDFDIDVNASVFETNIRVVGGLLSAHLLSKKAGVEVEAGWPCSGPLLRMAEEAARKLLPAFQTPTGMPYGTVNLLHGVNPGETPVTCTAGIGTFIVEFATLSSLTGDPVFEDVARXALMRLWESRSDIGLVGNHIDVLTGKWVAQDAGIGAGVDSYFEYLVKGAILLQDKKLMAMFLEYNXAIRNYTXFDDWYLWVQMYKGTVSMPVFQSLEAYWPGLQSLIGDIDNAMRTFLNYYTVWKQFGGLPEFYNIXQGYTVEKREGYPLRPELIESAMYLYRATGDPTLLELGRDAVESIEKISKVECGFATIKDLRDHKLDNRMESFFLAETVKYLYLLFXPXNFIHNNGSTFDXVXTPXGECILGAGGYIFNTEAHPIDPAALHCCXRLKEEQWEVEDLXXEXXSLXXSRXXXXQXXTVXSGPWEPXXXPXXXXXPXXXXQXREXXPAXQXXPLLSCPSQPFTSKLALLGQVFLDSS

SEQ ID NO: 9 - protein, 371 aa, Mus musculus
MVVVAAAPSAATAAPKVLLLSGQPASGGRALPLMVPGPRAAGSEASGTPQARKRQRLTHLSPEEKALRRKLKNRVAAQTARDRKKARMSELEQQVVDLEEENHKLQLENQLLREKTHGLVVENQELRTRLGMDTLDPDEVPEVEAKGSGVRLVAGSAESAAGAGPVVTSPEHLPMDSDTVASSDSESDILLGILDKLDPVMFFKCPSPESASLEELPEVYPEGPSSLPASLSLSVGTSSAKLEAINELIRFDHVYTKPLVLEIPSETESQTNVVVKIEEAPLSSSEEDHPEFIVSVKKEPLEDDFIPELGISNLLSSSHCLRPPSCLLDAHSDCGYEGSPSPFSDMSSPLGTDHSWEDTFANELFPQLISV

SEQ ID NO: 10 - protein, 369 aa, Cricetulus griseus
MVVVAASPSAATAAPKVLLLSGQPAADGRALPLMVPGSRAAGSEANGAPQARKRQRLTHLSPEEKALRRKLKNRVAAQTARDRKKARMSELEQQVVDLEEENQKLLLENQLLREKTHGLVIENQELRTRLGMDVLTTEEAPETESKGNGVRPVAGSAESAAGAGPVVTSPEHLPMDSDTVDSSDSESDILLGILDKLDPVMFFKCPSPESANLEELPEVYPGPSSLPASLSLSVGTSSAKLEAINELIRFDHVYTKPLVLEIPSETESQTNVVVKIEEAPLSSSEEDHPEFIVSVKKEPEEDFIPEPGISNLLSSSHCLKPSSCLLDAYSDCGYEGSPSPFSDMSSPLGIDHSWEDTFANELFPQLISV

SEQ ID NO: 11 - protein, 376 aa, Homo sapiens
MVVVAAAPNPADGTPKVLLLSGQPASAAGAPAGQALPLMVPAQRGASPEAASGGLPQARKRQRLTHLSPEEKALRRKLKNRVAAQTARDRKKARMSELEQQVVDLEEENQKLLLENQLLREKTHGLVVENQELRQRLGMDALVAEEEAEAKGNEVRPVAGSAESAAGAGPVVTPPEHLPMDSGGIDSSDSESDILLGILDNLDPVMFFKCPSPEPASLEELPEVYPEGPSSLPASLSLSVGTSSAKLEAINELIRFDHIYTKPLVLEIPSETESQANVVVKIEEAPLSPSENDHPEFIVSVKEEPVEDDLVPELGISNLLSSSHCPKPSSCLLDAYSDCGYGGSLSPFSDMSSLLGVNHSWEDTFANELFPQLISV

SEQ ID NO: 12 - protein, 383 aa, Danio rerio
MVVVTAGTGGAHKVLLISGKQSASTGATQGGYSRSISVMIPNQASSDSDSTTSGPPLRKRQRLTHLSPEEKALRRKLKNRVAAQTARDRKKAKMGELEQQVLELELENQKLHVENRLLRDKTSDLLSENEELRQRLGLDTLETKEQVQVLESAVSDLGLVTGSSESAAGAGPAVPKSEDFTMDTHSPGPADSESDLLLGILDILDPELFLKTDLPEAQEPQQELVLVGGAGEQVPSSAPAALGPAPVKLEALNELIHFDHIYTKPAEVLVSEESICEVKAEDSVAFSETEEEIQVEDQTVSVKDEPEEVVIPAENQNPDAADDFLSDTSFGGYEKASYLTDAYSDSGYERSPSPFSNISSPLCSEGSWDDMFASELFPQLISV

SEQ ID NO: 13 - protein, 373 aa, synthetic construct
  REGION 1..373: note = consensus sequence
  SITE 7: note = MISC_FEATURE - A or S
  SITE 9: note = MISC_FEATURE - S or N
  SITE 10: note = MISC_FEATURE - A or P
  SITE 12: note = MISC_FEATURE - T or D
  SITE 13: note = MISC_FEATURE - A or G
  SITE 14: note = MISC_FEATURE - A or T
  SITE 26: note = MISC_FEATURE - S or A
  SITE 27: note = MISC_FEATURE - G, D, or A
  SITE 29: note = MISC_FEATURE - R or Q
  SITE 37: note = MISC_FEATURE - G or A
  SITE 38: note = misc_feature - Xaa can be any naturally occurring amino acid
  SITE 40: note = MISC_FEATURE - A or G
  REGION 46..48: note = MISC_FEATURE - S, N, or ASG (two amino acids may be missing)
  SITE 50: note = MISC_FEATURE - T, A, or L
  SITE 105: note = MISC_FEATURE - H or Q
  SITE 108: note = MISC_FEATURE - Q or L
  SITE 123: note = MISC_FEATURE - V or I
  SITE 130: note = MISC_FEATURE - T or Q
  SITE 136: note = MISC_FEATURE - T, V, or A
  SITE 138: note = MISC_FEATURE - D, T, or V
  SITE 139: note = MISC_FEATURE - P, T, or A
  SITE 140: note = MISC_FEATURE - D or E
  SITE 142: note = MISC_FEATURE - V, A, or none
  SITE 143: note = MISC_FEATURE - P or none
  SITE 145: note = MISC_FEATURE - V, T, or A
  SITE 147: note = MISC_FEATURE - A or S
  SITE 150: note = MISC_FEATURE - S or N
  SITE 151: note = MISC_FEATURE - G or E
  SITE 154: note = MISC_FEATURE - L or P
  SITE 171: note = MISC_FEATURE - S or P
  SITE 180: note = MISC_FEATURE - D or G
  SITE 181: note = MISC_FEATURE - T or G
  SITE 182: note = MISC_FEATURE - V or I
  SITE 183: note = MISC_FEATURE - A or D
  SITE 198: note = MISC_FEATURE - K or N
  SITE 212: note = MISC_FEATURE - S or P
  SITE 214: note = MISC_FEATURE - S or N
  SITE 224: note = MISC_FEATURE - E or none
  SITE 256: note = MISC_FEATURE - V or I
  SITE 273: note = MISC_FEATURE - T or A
  SITE 286: note = MISC_FEATURE - S or P
  SITE 289: note = MISC_FEATURE - E or N
  SITE 300: note = MISC_FEATURE - K or E
  SITE 303: note = MISC_FEATURE - L, V, or none
  SITE 305: note = MISC_FEATURE - D or E
  SITE 307: note = MISC_FEATURE - F or L
  SITE 308: note = MISC_FEATURE - I or V
  SITE 311: note = MISC_FEATURE - L or P
  SITE 323: note = MISC_FEATURE - L or P
  SITE 324: note = MISC_FEATURE - R or K
  SITE 326: note = MISC_FEATURE - P or S
  SITE 333: note = MISC_FEATURE - H or Y
  SITE 339: note = MISC_FEATURE - E or G
  SITE 342: note = MISC_FEATURE - P or L
  SITE 351: note = MISC_FEATURE - P or L
  SITE 354: note = MISC_FEATURE - T, I, or V
  SITE 355: note = MISC_FEATURE - D or N
MVVVAAXPXXAXXXPKVLLLSGQPAXXGXALPLMVPXXRXAGSEAXXXGXPQARKRQRLTHLSPEEKALRRKLKNRVAAQTARDRKKARMSELEQQVVDLEEENXKLXLENQLLREKTHGLVXENQELRXRLGMDXLXXXEXXEXEXKGXXVRXVAGSAESAAGAGPVVTXPEHLPMDSXXXXSSDSESDILLGILDXLDPVMFFKCPSPEXAXLEELPEVYPXGPSSLPASLSLSVGTSSAKLEAINELIRFDHXYTKPLVLEIPSETESQXNVVVKIEEAPLSXSEXDHPEFIVSVKXEPXEXDXXPEXGISNLLSSSHCXXPXSCLLDAXSDCGYXGSXSPFSDMSSXLGXXHSWEDTFANELFPQLISV

SEQ ID NO: 14 - DNA, 7686 bp, synthetic construct
  misc_feature 1..7686: note = Synthetic plasmid
  source 1..7686: mol_type = other DNA
aagcttatactcgagctctagattgggaacccgggtctctcgaattcgatgccttttagactcctgataccattgggtcttgtttgcgttctcctccctctccatcacggcgccccaggtccagacggtaccgcacctgatcctgcccattaccgcgaacgcgttaaagccatgttctaccacgcctatgactcctatctggaaaatgcattcccctatgatgagctccgaccccttacctgcgatggtcatgatacttggggctctttttcccttacccttattgacgctctggacacactccttatcctcggaaacaccagcgaatttcaaagagtagttgaagtacttcaggacaatgtcgactttgacatcgatgtgaacgcatcagttttcgaaacaaatataagagtcgttggaggtctgctctccgcccaccttctctctaaaaaagccggagtagaagttgaagctggctggccctgctccggacccctccttcgtatggctgaagaagctgcccgcaaactccttcccgcttttcagaccccaaccggtatgccctatggtactgttaacctcctgcacggagtaaatcccggcgaaacccccgtcacatgtacagccggaattggaacctttattgtggaatttgcaacccttagcagcctgaccggagatcctgtattcgaagacgtggctcgggttgccctgatgcgactgtgggaatccaggtctgatatcggtctggtcggtaaccatatagacgtactcactggtaaatgggttgcacaagacgctggaattggggcaggcgtggattcttattttgaatatctcgtaaaaggggccatactcttgcaggacaaaaaacttatggctatgttcctggaatataacaaagctattaggaactacacacacttcgatgattggtatttgtgggtccaaatgtataaaggaaccgtttctatgcctgtctttcagtcactggaggcttattggcctggtctgcaatccctgatcggagacattgacaatgcaatgaggacattccttaattattacactgtttggaagcagttcggcggattgcccgaattttacaacattcctcaaggctatacagttgaaaaaagagaaggatatcccctgcgccccgagcttattgaaagcgctatgtatctgtatcgtgcaacaggtgatccaaccctgcttgaactgggacgagacgccgtcgaatcaatcgagaaaatttcaaaagtggaatgcggctttgcaacaattaaagatcttagagaccacaaactggataatcgcatggagtcattctttttggctgagaccgtcaagtatctgtatctgctttttcatcccaacaacttcatccataataacgggtccaccttcgattcagtcatgacccctcacggtgaatgcatactcggagctggaggctatatttttaacactgaagctcacccaattgacccagctgcccttcattgttgtcgacgtctgaaagaagaacaatgggaggttgaagatttgatcaaagaattttactcacttaaacaaagtcgacctaaacgcgcacagagaaaaactgtaagatctggtccttgggaacctcagtccggcccagcaactctttcatcccccgccaaccaaccacgagaaaaacaaccagcccaacagagaacccccctgctcagctgcccctctcagcccttcacttcaaaactcgccctgcttggacaggtgtttctggactcctcttgatttaaacacgcggccgctaatcagccataccacatttgtagaggttttacttgctttaaaaaacctcccacacctccccctgaacctgaaacataaaatgaatgcaattgttgttgttaacttgtttattgcagcttataatggttacaaataaagcaatagcatcacaaatttcacaaataaagcatttttttcactgcattctagttgtggtttgtccaaactcatcaatgtatcttatcatgtctaccggtagggcccctctcttcatgtgagcaaaaggccagcaaaaggccaggaaccgtaaaaaggccgcgttgctggcgtttttccataggctccgcccccctgacgagcatcacaaaaatcgacgctcaagtcagaggtggcgaaacccgacaggactataaagataccaggcgtttccccctggaagctccctcgtgcgctctcctgttccgaccctgccgcttaccggatacctgtccgcctttctcccttcgggaagcgtggcgctttctcaatgctcacgctgtaggtatctcagttcggtgtaggtcgttcgctccaagctgggctgtgtgcacgaaccccccgttcagcccgaccgctgcgccttatccggtaactatcgtcttgagtccaacccggtaagacacgacttatcgccactggcagcagccactggtaacaggattagcagagcgaggtatgtaggcggtgctacagagttcttgaagtggtggcctaactacggctacactagaaggacagtatttggtatctgcgctctgctgaagccagttaccttcggaaaaagagttggtagctcttgatccggcaaacaaaccaccgctggtagcggtggtttttttgtttgcaagcagcagattacgcgcagaaaaaaaggatctcaagaagatcctttgatcttttctacggggtctgacgctcagtggaacgaaaactcacgttaagggattttggtcatgggcgcgcctcatactcctgcaggcatgagattatcaaaaaggatcttcacctagatccttttaaattaaaaatgaagttttaaatcaatctaaagtatatatgagtaaacttggtctgacagttaccaatgcttaatcagtgaggcacctatctcagcgatctgtctatttcgttcatccatagttgcctgactccccgtcgtgtagataactacgatacgggagggcttaccatctggccccagtgctgcaatgataccgcgagacccacgctcaccggctccagatttatcagcaataaaccagccagccggaagggccgagcgcagaagtggtcctgcaactttatccgcctccatccagtctattaattgttgccgggaagctagagtaagtagttcgccagttaatagtttgcgcaacgttgttgccattgctacaggcatcgtggtgtcacgctcgtcgtttggtatggcttcattcagctccggttcccaacgatcaaggcgagttacatgatcccccatgttgtgcaaaaaagcggttagctccttcggtcctccgatcgttgtcagaagtaagttggccgcagtgttatcactcatggttatggcagcactgcataattctcttactgtcatgccatccgtaagatgcttttctgtgactggtgagtactcaaccaagtcattctgagaatagtgtatgcggcgaccgagttgctcttgcccggcgtcaatacgggataataccgcgccacatagcagaactttaaaagtgctcatcattggaaaacgttcttcggggcgaaaactctcaaggatcttaccgctgttgagatccagttcgatgtaacccactcgtgcacccaactgatcttcagcatcttttactttcaccagcgtttctgggtgagcaaaaacaggaaggcaaaatgccgcaaaaaagggaataagggcgacacggaaatgttgaatactcatactcttcctttttcaatattattgaagcatttatcagggttattgtctcatgagcggatacatatttgaatgtatttagaaaaataaacaaataggggttccgcgcacatttccccgaaaagtgccacctgacgtcaggtaccaagcctaggcctccaaaaaagcctcctcactacttctggaatagctcagaggcagaggcggcctcggcctctgcataaataaaaaaaattagtcagccatggggcggagaatgggcggaactgggcggagttaggggcgggatgggcggagttaggggcgggactatggttgctgactaattgagatgcatgctttgcatacttctgcctgctggggagcctggggactttccacacctggttgctgactaattgagatgcatgctttgcatacttctgcctgctggggagcctggggactttccacaccggatccaccatgggatcggccattgaacaagatggattgcacgcaggttctccggccgcttgggtggagaggctattcggctatgactgggcacaacagacaatcggctgctctgatgccgccgtgttccggctgtcagcgcaggggcgcccggttctttttgtcaagaccgacctgtccggtgccctgaatgaactgcaggacgaggcagcgcggctatcgtggctggccacgacgggcgttccttgcgcagctgtgctcgacgttgtcactgaagcgggaagggactggctgctattgggcgaagtgccggggcaggatctcctgtcatctcaccttgctcctgccgagaaagtatccatcatggctgatgcaatgcggcggctgcatacgcttgatccggctacctgcccattcgaccaccaagcgaaacatcgcatcgagcgagcacgtactcggatggaagccggtcttgtcgatcaggatgatctggacgaagagcatcaggggctcgcgccagccgaactgttcgccaggctcaaggcgcgcatgcccgacggcgatgatctcgtcgtgacccatggcgatgcctgcttgccgaatatcatggtggaaaatggccgcttttctggattcatcgactgtggccggctgggtgtggcggaccgctatcaggacatagcgttggctacccgtgatattgctgaagagcttggcggcgaatgggctgaccgcttcctcgtgctttacggtatcgccgctcccgattcgcagcgcatcgccttctatcgccttcttgacgagttcttctgaacgcgtgctgtaagtctgcagaaattgatgatctattaaacaataaagatgtccactaaaatggaagtttttcctgtcatactttgttaagaagggtgagaacagagtacctacattttgaatggaaggattggagctacgggggtgggggtggggtgggattagataaatgcctgctctttactgaaggctctttactattgctttatgataatgtttcatagttggatatcataatttaaacaagcaaaaccaaattaagggccagctcattcctcccactcatgatctatggatctatagatctctcgtgcagctggggctctagggggtatccccacgcgccctgtagcggcgcattaagcgcggcgggtgtggtggttacgcgcagcgtgaccgctacacttgccagcgccctagcgcccgctcctttcgctttcttcccttcctttctcgccacgttcgccggctttccccgtcaagctctaaatcgggggctccctttagggttccgatttagtgctttacggcacctcgaccccaaaaaacttgattagggtgatggttcacgtagtgggccatcgccctgatagacggtttttcgccctttgacgttggagtccacgttctttaatagtggactcttgttccaaactggaacaacactcaaccctatctcggtctattcttttgatttataagggattttgccgatttcggcctattggttaaaaaatgagctgatttaacaaaaatttaacgcgaattaattctgtggaatgtgtgtcagttagtcgcgaggcctccgcgccgggttttggcgcctcccgcgggcgcccccctcctcacggcgagcgctgccacgtcagacgaagggcgcagcgagcgtcctgatccttccgcccggacgctcaggacagcggcccgctgctcataagactcggccttagaaccccagtatcagcagaaggacattttaggacgggacttgggtgactctagggcactggttttctttccagagagcggaacaggcgaggaaaagtagtcccttctcggcgattctgcggagggatctccgtggggcggtgaacgccgatgattatataaggacgcgccgggtgtggcacagctagttccgtcgcagccgggatttgggtcgcggttcttgtttgtggatcgctgtgatcgtcacttggtgagtagcgggctgctgggctggccggggctttcgtggccgccgggccgctcggtgggacggaagcgtgtggagagaccgccaagggctgtagtctgggtccgcgagcaaggttgccctgaactgggggttggggggagcgcagcaaaatggcggctgttcccgagtcttgaatggaagacgcttgtgaggcgggctgtgaggtcgttgaaacaaggtggggggcatggtgggcggcaagaacccaaggtcttgaggccttcgctaatgcgggaaagctcttattcgggtgagatgggctggggcaccatctggggaccctgacgtgaagtttgtcactgactggagaactcggtttgtcgtctgttgcgggggcggcagttatggcggtgccgttgggcagtgcacccgtacctttgggagcgcgcgccctcgtcgtgtcgtgacgtcacccgttctgttggcttataatgcagggtggggccacctgccggtaggtgtgcggtaggcttttctccgtcgcaggacgcagggttcgggcctagggtaggctctcctgaatcgacaggcgccggacctctggtgaggggagggataagtgaggcgtcagtttctttggtcggttttatgtacctatcttcttaagtagctgaagctccggttttgaactatgcgctcggggttggcgagtgtgttttgtgaagttttttaggcaccttttgaaatgtaatcatttgggtcaatatgtaattttcagtgttagactagtaaattgtccgctaaattctggccgtttttggcttttttgttagacgtcgaccgatcctgagaacttcagggtgagtttggggacccttgattgttctttctttttcgctattgtaaaattcatgttatatggagggggcaaagttttcagggtgttgtttagaatgggaagatgtcccttgtatcaccatggaccctcatgataattttgtttctttcactttctactctgttgacaaccattgtctcctcttattttcttttcattttctgtaactttttcgttaaactttagcttgcatttgtaacgaatttttaaattcacttttgtttatttgtcagattgtaagtactttctctaatcacttttttttcaaggcaatcagggtatattatattgtacttcagcacagttttagagaacaattgttataattaaatgataaggtagaatatttctgcatataaattctggctggcgtggaaatattcttattggtagaaacaactacaccctggtcatcatcctgcctttctctttatggttacaatgatatacactgtttgagatgaggataaaatactctgagtccaaaccgggcccctctgctaaccatgttcatgccttcttctctttcctacagctcctgggcaacgtgctggttgttgtgctgtctcatcattttggcaaagaatt

SEQ ID NO: 15 - DNA, 7257 bp, synthetic construct
  misc_feature 1..7257: note = Synthetic plasmid
  source 1..7257: mol_type = other DNA
aagcttatactcgagctctagattgggaacccgggtctctcgaattcgatgccttttagactcctgataccattgggtcttgtttgcgttctcctccctctccatcacggcgccccaggtccagacggtaccgcacctgatcctgcccattaccgcgaacgcgttaaagccatgttctaccacgcctatgactcctatctggaaaatgcattcccctatgatgagctccgaccccttacctgcgatggtcatgatacttggggctctttttcccttacccttattgacgctctggacacactccttatcctcggaaacaccagcgaatttcaaagagtagttgaagtacttcaggacaatgtcgactttgacatcgatgtgaacgcatcagttttcgaaacaaatataagagtcgttggaggtctgctctccgcccaccttctctctaaaaaagccggagtagaagttgaagctggctggccctgctccggacccctccttcgtatggctgaagaagctgcccgcaaactccttcccgcttttcagaccccaaccggtatgccctatggtactgttaacctcctgcacggagtaaatcccggcgaaacccccgtcacatgtacagccggaattggaacctttattgtggaatttgcaacccttagcagcctgaccggagatcctgtattcgaagacgtggctcgggttgccctgatgcgactgtgggaatccaggtctgatatcggtctggtcggtaaccatatagacgtactcactggtaaatgggttgcacaagacgctggaattggggcaggcgtggattcttattttgaatatctcgtaaaaggggccatactcttgcaggacaaaaaacttatggctatgttcctggaatataacaaagctattaggaactacacacacttcgatgattggtatttgtgggtccaaatgtataaaggaaccgtttctatgcctgtctttcagtcactggaggcttattggcctggtctgcaatccctgatcggagacattgacaatgcaatgaggacattccttaattattacactgtttggaagcagttcggcggattgcccgaattttacaacattcctcaaggctatacagttgaaaaaagagaaggatatcccctgcgccccgagcttattgaaagcgctatgtatctgtatcgtgcaacaggtgatccaaccctgcttgaactgggacgagacgccgtcgaatcaatcgagaaaatttcaaaagtggaatgcggctttgcaacaattaaagatcttagagaccacaaactggataatcgcatggagtcattctttttggctgagaccgtcaagtatctgtatctgctttttcatcccaacaacttcatccataataacgggtccaccttcgattcagtcatgacccctcacggtgaatgcatactcggagctggaggctatatttttaacactgaagctcacccaattgacccagctgcccttcattgttgtcgacgtctgaaagaagaacaatgggaggttgaagatttgatcaaagaattttactcacttaaacaaagtcgacctaaacgcgcacagagaaaaactgtaagatctggtccttgggaacctcagtccggcccagcaactctttcatcccccgccaaccaaccacgagaaaaacaaccagcccaacagagaacccccctgctcagctgcccctctcagcccttcacttcaaaactcgccctgcttggacaggtgtttctggactcctcttgatttaaacacgcggccgctaatcagccataccacatttgtagaggttttacttgctttaaaaaacctcccacacctccccctgaacctgaaacataaaatgaatgcaattgttgttgttaacttgtttattgcagcttataatggttacaaataaagcaatagcatcacaaatttcacaaataaagcatttttttcactgcattctagttgtggtttgtccaaactcatcaatgtatcttatcatgtctaccggtagggcccctctcttcatgtgagcaaaaggccagcaaaaggccaggaaccgtaaaaaggccgcgttgctggcgtttttccataggctccgcccccctgacgagcatcacaaaaatcgacgctcaagtcagaggtggcgaaacccgacaggactataaagataccaggcgtttccccctggaagctccctcgtgcgctctcctgttccgaccctgccgcttaccggatacctgtccgcctttctcccttcgggaagcgtggcgctttctcatagctcacgctgtaggtatctcagttcggtgtaggtcgttcgctccaagctgggctgtgtgcacgaaccccccgttcagcccgaccgctgcgccttatccggtaactatcgtcttgagtccaacccggtaagacacgacttatcgccactggcagcagccactggtaacaggattagcagagcgaggtatgtaggcggtgctacagagttcttgaagtggtggcctaactacggctacactagaaggacagtatttggtatctgcgctctgctgaagccagttaccttcggaaaaagagttggtagctcttgatccggcaaacaaaccaccgctggtagcggtggtttttttgtttgcaagcagcagattacgcgcagaaaaaaaggatctcaagaagatcctttgatcttttctacggggtctgacgctcagtggaacgaaaactcacgttaagggattttggtcatgggcgcgcctcatactcctgcaggcatgagattatcaaaaaggatcttcacctagatccttttaaattaaaaatgaagttttaaatcaatctaaagtatatatgagtaaacttggtctgacagttaccaatgcttaatcagtgaggcacctatctcagcgatctgtctatttcgttcatccatagttgcctgactccccgtcgtgtagataactacgatacgggagggcttaccatctggccccagtgctgcaatgataccgcgagacccacgctcaccggctccagatttatcagcaataaaccagccagccggaagggccgagcgcagaagtggtcctgcaactttatccgcctccatccagtctattaattgttgccgggaagctagagtaagtagttcgccagttaatagtttgcgcaacgttgttgccattgctacaggcatcgtggtgtcacgctcgtcgtttggtatggcttcattcagctccggttcccaacgatcaaggcgagttacatgatcccccatgttgtgcaaaaaagcggttagctccttcggtcctccgatcgttgtcagaagtaagttggccgcagtgttatcactcatggttatggcagcactgcataattctcttactgtcatgccatccgtaagatgcttttctgtgactggtgagtactcaaccaagtcattctgagaatagtgtatgcggcgaccgagttgctcttgcccggcgtcaatacgggataataccgcgccacatagcagaactttaaaagtgctcatcattggaaaacgttcttcggggcgaaaactctcaaggatcttaccgctgttgagatccagttcgatgtaacccactcgtgcacccaactgatcttcagcatcttttactttcaccagcgtttctgggtgagcaaaaacaggaaggcaaaatgccgcaaaaaagggaataagggcgacacggaaatgttgaatactcatactcttcctttttcaatattattgaagcatttatcagggttattgtctcatgagcggatacatatttgaatgtatttagaaaaataaacaaataggggttccgcgcacatttccccgaaaagtgccacctgacgtcaggtaccaagcctaggcctccaaaaaagcctcctcactacttctggaatagctcagaggcagaggcggcctcggcctctgcataaataaaaaaaattagtcagccatggggcggagaatgggcggaactgggcggagttaggggcgggatgggcggagttaggggcgggactatggttgctgactaattgagatgcatgctttgcatacttctgcctgctggggagcctggggactttccacacctggttgctgactaattgagatgcatgctttgcatacttctgcctgctggggagcctggggactttccacaccggatccaccatggccaagttgaccagtgccgttccggtgctcaccgcgcgcgacgtcgccggagcggtcgagttctggaccgaccggctcgggttctcccgggacttcgtggaggacgacttcgccggtgtggtccgggacgacgtgaccctgttcatcagcgcggtccaggaccaggtggtgccggacaacaccctggcctgggtgtgggtgcgcggcctggacgagctgtacgccgagtggtcggaggtcgtgtccacgaacttccgggacgcctccgggccggccatgaccgagatcggcgagcagccgtgggggcgggagttcgccctgcgcgacccggccggcaactgcgtgcacttcgtggccgaggagcaggactgaacgcgtgctgtaagtctgcagaaattgatgatctattaaacaataaagatgtccactaaaatggaagtttttcctgtcatactttgttaagaagggtgagaacagagtacctacattttgaatggaaggattggagctacgggggtgggggtggggtgggattagataaatgcctgctctttactgaaggctctttactattgctttatgataatgtttcatagttggatatcataatttaaacaagcaaaaccaaattaagggccagctcattcctcccactcatgatctatggatctatagatctctcgtgcagctggggctctagggggtatccccacgcgccctgtagcggcgcattaagcgcggcgggtgtggtggttacgcgcagcgtgaccgctacacttgccagcgccctagcgcccgctcctttcgctttcttcccttcctttctcgccacgttcgccggctttccccgtcaagctctaaatcgggggctccctttagggttccgatttagtgctttacggcacctcgaccccaaaaaacttgattagggtgatggttcacgtagtgggccatcgccctgatagacggtttttcgccctttgacgttggagtccacgttctttaatagtggactcttgttccaaactggaacaacactcaaccctatctcggtctattcttttgatttataagggattttgccgatttcggcctattggttaaaaaatgagctgatttaacaaaaatttaacgcgaattaattctgtggaatgtgtgtcagttagtcgcgaggcctccgcgccgggttttggcgcctcccgcgggcgcccccctcctcacggcgagcgctgccacgtcagacgaagggcgcagcgagcgtcctgatccttccgcccggacgctcaggacagcggcccgctgctcataagactcggccttagaaccccagtatcagcagaaggacattttaggacgggacttgggtgactctagggcactggttttctttccagagagcggaacaggcgaggaaaagtagtcccttctcggcgattctgcggagggatctccgtggggcggtgaacgccgatgattatataaggacgcgccgggtgtggcacagctagttccgtcgcagccgggatttgggtcgcggttcttgtttgtggatcgctgtgatcgtcacttggtgagtagcgggctgctgggctggccggggctttcgtggccgccgggccgctcggtgggacggaagcgtgtggagagaccgccaagggctgtagtctgggtccgcgagcaaggttgccctgaactgggggttggggggagcgcagcaaaatggcggctgttcccgagtcttgaatggaagacgcttgtgaggcgggctgtgaggtcgttgaaacaaggtggggggcatggtgggcggcaagaacccaaggtcttgaggccttcgctaatgcgggaaagctcttattcgggtgagatgggctggggcaccatctggggaccctgacgtgaagtttgtcactgactggagaactcggtttgtcgtctgttgcgggggcggcagttatggcggtgccgttgggcagtgcacccgtacctttgggagcgcgcgccctcgtcgtgtcgtgacgtcacccgttctgttggcttataatgcagggtggggccacctgccggtaggtgtgcggtaggcttttctccgtcgcaggacgcagggttcgggcctagggtaggctctcctgaatcgacaggcgccggacctctggtgaggggagggataagtgaggcgtcagtttctttggtcggttttatgtacctatcttcttaagtagctgaagctccggttttgaactatgcgctcggggttggcgagtgtgttttgtgaagttttttaggcaccttttgaaatgtaatcatttgggtcaatatgtaattttcagtgttagactagtaaattgtccgctaaattctggccgtttttggcttttttgttagacgtcgaccgatcctgagaacttcagggtgagtttggggacccttgattgttctttctttttcgctattgtaaaattcatgttatatggagggggcaaagttttcagggtgttgtttagaatgggaagatgtcccttgtatcaccatggaccctcatgataattttgtttctttcactttctactctgttgacaaccattgtctcctcttattttcttttcattttctgtaactttttcgttaaactttagcttgcatttgtaacgaatttttaaattcacttttgtttatttgtcagattgtaagtactttctctaatcacttttttttcaaggcaatcagggtatattatattgtacttcagcacagttttagagaacaattgttataattaaatgataaggtagaatatttctgcatataaattctggctggcgtggaaatattcttattggtagaaacaactacaccctggtcatcatcctgcctttctctttatggttacaatgatatacactgtttgagatgaggataaaatactctgagtccaaaccgggcccctctgctaaccatgttcatgccttcttctctttcctacagctcctgggcaacgtgctggttgttgtgctgtctcatcattttggcaaagaatt

SEQ ID NO: 16 - DNA, 3892 bp, synthetic construct
  misc_feature 1..3892: note = Synthetic construct
  source 1..3892: mol_type = other DNA
aggcctccgcgccgggttttggcgcctcccgcgggcgcccccctcctcacggcgagcgctgccacgtcagacgaagggcgcagcgagcgtcctgatccttccgcccggacgctcaggacagcggcccgctgctcataagactcggccttagaaccccagtatcagcagaaggacattttaggacgggacttgggtgactctagggcactggttttctttccagagagcggaacaggcgaggaaaagtagtcccttctcggcgattctgcggagggatctccgtggggcggtgaacgccgatgattatataaggacgcgccgggtgtggcacagctagttccgtcgcagccgggatttgggtcgcggttcttgtttgtggatcgctgtgatcgtcacttggtgagtagcgggctgctgggctggccggggctttcgtggccgccgggccgctcggtgggacggaagcgtgtggagagaccgccaagggctgtagtctgggtccgcgagcaaggttgccctgaactgggggttggggggagcgcagcaaaatggcggctgttcccgagtcttgaatggaagacgcttgtgaggcgggctgtgaggtcgttgaaacaaggtggggggcatggtgggcggcaagaacccaaggtcttgaggccttcgctaatgcgggaaagctcttattcgggtgagatgggctggggcaccatctggggaccctgacgtgaagtttgtcactgactggagaactcggtttgtcgtctgttgcgggggcggcagttatggcggtgccgttgggcagtgcacccgtacctttgggagcgcgcgccctcgtcgtgtcgtgacgtcacccgttctgttggcttataatgcagggtggggccacctgccggtaggtgtgcggtaggcttttctccgtcgcaggacgcagggttcgggcctagggtaggctctcctgaatcgacaggcgccggacctctggtgaggggagggataagtgaggcgtcagtttctttggtcggttttatgtacctatcttcttaagtagctgaagctccggttttgaactatgcgctcggggttggcgagtgtgttttgtgaagttttttaggcaccttttgaaatgtaatcatttgggtcaatatgtaattttcagtgttagactagtaaattgtccgctaaattctggccgtttttggcttttttgttagacgtcgaccgatcctgagaacttcagggtgagtttggggacccttgattgttctttctttttcgctattgtaaaattcatgttatatggagggggcaaagttttcagggtgttgtttagaatgggaagatgtcccttgtatcaccatggaccctcatgataattttgtttctttcactttctactctgttgacaaccattgtctcctcttattttcttttcattttctgtaactttttcgttaaactttagcttgcatttgtaacgaatttttaaattcacttttgtttatttgtcagattgtaagtactttctctaatcacttttttttcaaggcaatcagggtatattatattgtacttcagcacagttttagagaacaattgttataattaaatgataaggtagaatatttctgcatataaattctggctggcgtggaaatattcttattggtagaaacaactacaccctggtcatcatcctgcctttctctttatggttacaatgatatacactgtttgagatgaggataaaatactctgagtccaaaccgggcccctctgctaaccatgttcatgccttcttctctttcctacagctcctgggcaacgtgctggttgttgtgctgtctcatcattttggcaaagaattaagcttatactcgagctctagattgggaacccgggtctctcgaattcgatgccttttagactcctgataccattgggtcttgtttgcgttctcctccctctccatcacggcgccccaggtccagacggtaccgcacctgatcctgcccattaccgcgaacgcgttaaagccatgttctaccacgcctatgactcctatctggaaaatgcattcccctatgatgagctccgaccccttacctgcgatggtcatgatacttggggctctttttcccttacccttattgacgctctggacacactccttatcctcggaaacaccagcgaatttcaaagagtagttgaagtacttcaggacaatgtcgactttgacatcgatgtgaacgcatcagttttcgaaacaaatataagagtcgttggaggtctgctctccgcccaccttctctctaaaaaagccggagtagaagttgaagctggctggccctgctccggacccctccttcgtatggctgaagaagctgcccgcaaactccttcccgcttttcagaccccaaccggtatgccctatggtactgttaacctcctgcacggagtaaatcccggcgaaacccccgtcacatgtacagccggaattggaacctttattgtggaatttgcaacccttagcagcctgaccggagatcctgtattcgaagacgtggctcgggttgccctgatgcgactgtgggaatccaggtctgatatcggtctggtcggtaaccatatagacgtactcactggtaaatgggttgcacaagacgctggaattggggcaggcgtggattcttattttgaatatctcgtaaaaggggccatactcttgcaggacaaaaaacttatggctatgttcctggaatataacaaagctattaggaactacacacacttcgatgattggtatttgtgggtccaaatgtataaaggaaccgtttctatgcctgtctttcagtcactggaggcttattggcctggtctgcaatccctgatcggagacattgacaatgcaatgaggacattccttaattattacactgtttggaagcagttcggcggattgcccgaattttacaacattcctcaaggctatacagttgaaaaaagagaaggatatcccctgcgccccgagcttattgaaagcgctatgtatctgtatcgtgcaacaggtgatccaaccctgcttgaactgggacgagacgccgtcgaatcaatcgagaaaatttcaaaagtggaatgcggctttgcaacaattaaagatcttagagaccacaaactggataatcgcatggagtcattctttttggctgagaccgtcaagtatctgtatctgctttttcatcccaacaacttcatccataataacgggtccaccttcgattcagtcatgacccctcacggtgaatgcatactcggagctggaggctatatttttaacactgaagctcacccaattgacccagctgcccttcattgttgtcgacgtctgaaagaagaacaatgggaggttgaagatttgatcaaagaattttactcacttaaacaaagtcgacctaaacgcgcacagagaaaaactgtaagatctggtccttgggaacctcagtccggcccagcaactctttcatcccccgccaaccaaccacgagaaaaacaaccagcccaacagagaacccccctgctcagctgcccctctcagcccttcacttcaaaactcgccctgcttggacaggtgtttctggactcctcttgatttaaacacgcggccgctaatcagccataccacatttgtagaggttttacttgctttaaaaaacctcccacacctccccctgaacctgaaacataaaatgaatgcaattgttgttgttaacttgtttattgcagcttataatggttacaaataaagcaatagcatcacaaatttcacaaataaagcatttttttcactgcattctagttgtggtttgtccaaactcatcaatgtatcttatcatgt

SEQ ID NO: 17 - DNA, 6629 bp, synthetic construct
  misc_feature 1..6629: note = Synthetic plasmid
  source 1..6629: mol_type = other DNA
aagcttatactcgagctctagattgggaacccgggtctctcgaattcatggtggtggtggctgctgctccttctgctgctacagctgctcctaaggtgctgctgctgtctggacagcctgcttctggaggaagagctctgcctctgatggtgcctggacctagagctgctggatctgaggcttctggaacacctcaggctagaaagagacagagactgacacatctgtctcctgaagaaaaggctctgagaagaaagctgaagaatagagtggctgctcagacagctagagatagaaagaaggctagaatgtctgaactggaacagcaggtggtggatctggaagaagaaaatcataagctgcagctggaaaatcagctgctgagagaaaagacacatggactggtggtggaaaatcaggaactgagaacaagactgggaatggatacactggatcctgatgaagtgcctgaagtggaagctaagggatctggagtgagactggtggctggatctgctgaatctgctgctggagctggacctgtggtgacatctcctgaacatctgcctatggattctgatacagtggcttcttctgattctgaatctgatatcctgctgggaatcctggataagctggatcctgtgatgttttttaagtgtccttctcctgaatctgcttctctggaagaactgcctgaagtgtatcctgaaggaccttcttctctgcctgcttctctgtctctgtctgtgggaacatcttctgctaagctggaagctatcaatgaactgatcagatttgatcatgtgtatacaaagcctctggtgctggaaatcccttctgaaacagaatctcagacaaatgtggtggtgaagatcgaagaagctcctctgtcttcttctgaagaagatcatcctgaatttatcgtgtctgtgaagaaggaacctctggaagatgattttatccctgaactgggaatctctaatctgctgtcttcttctcattgtctgagacctccttcttgtctgctggatgctcattctgattgtggatatgaaggatctccttctcctttttctgatatgtcttctcctctgggaacagatcattcttgggaagatacatttgctaatgaactgtttcctcagctgatctctgtgtgagcggccgctaatcagccataccacatttgtagaggttttacttgctttaaaaaacctcccacacctccccctgaacctgaaacataaaatgaatgcaattgttgttgttaacttgtttattgcagcttataatggttacaaataaagcaatagcatcacaaatttcacaaataaagcatttttttcactgcattctagttgtggtttgtccaaactcatcaatgtatcttatcatgtctaccggtagggcccctctcttcatgtgagcaaaaggccagcaaaaggccaggaaccgtaaaaaggccgcgttgctggcgtttttccataggctccgcccccctgacgagcatcacaaaaatcgacgctcaagtcagaggtggcgaaacccgacaggactataaagataccaggcgtttccccctggaagctccctcgtgcgctctcctgttccgaccctgccgcttaccggatacctgtccgcctttctcccttcgggaagcgtggcgctttctcatagctcacgctgtaggtatctcagttcggtgtaggtcgttcgctccaagctgggctgtgtgcacgaaccccccgttcagcccgaccgctgcgccttatccggtaactatcgtcttgagtccaacccggtaagacacgacttatcgccactggcagcagccactggtaacaggattagcagagcgaggtatgtaggcggtgctacagagttcttgaagtggtggcctaactacggctacactagaaggacagtatttggtatctgcgctctgctgaagccagttaccttcggaaaaagagttggtagctcttgatccggcaaacaaaccaccgctggtagcggtggtttttttgtttgcaagcagcagattacgcgcagaaaaaaaggatctcaagaagatcctttgatcttttctacggggtctgacgctcagtggaacgaaaactcacgttaagggattttggtcatgggcgcgcctcatactcctgcaggcatgagattatcaaaaaggatcttcacctagatccttttaaattaaaaatgaagttttaaatcaatctaaagtatatatgagtaaacttggtctgacagttaccaatgcttaatcagtgaggcacctatctcagcgatctgtctatttcgttcatccatagttgcctgactccccgtcgtgtagataactacgatacgggagggcttaccatctggccccagtgctgcaatgataccgcgagacccacgctcaccggctccagatttatcagcaataaaccagccagccggaagggccgagcgcagaagtggtcctgcaactttatccgcctccatccagtctattaattgttgccgggaagctagagtaagtagttcgccagttaatagtttgcgcaacgttgttgccattgctacaggcatcgtggtgtcacgctcgtcgtttggtatggcttcattcagctccggttcccaacgatcaaggcgagttacatgatcccccatgttgtgcaaaaaagcggttagctccttcggtcctccgatcgttgtcagaagtaagttggccgcagtgttatcactcatggttatggcagcactgcataattctcttactgtcatgccatccgtaagatgcttttctgtgactggtgagtactcaaccaagtcattctgagaatagtgtatgcggcgaccgagttgctcttgcccggcgtcaatacgggataataccgcgccacatagcagaactttaaaagtgctcatcattggaaaacgttcttcggggcgaaaactctcaaggatcttaccgctgttgagatccagttcgatgtaacccactcgtgcacccaactgatcttcagcatcttttactttcaccagcgtttctgggtgagcaaaaacaggaaggcaaaatgccgcaaaaaagggaataagggcgacacggaaatgttgaatactcatactcttcctttttcaatattattgaagcatttatcagggttattgtctcatgagcggatacatatttgaatgtatttagaaaaataaacaaataggggttccgcgcacatttccccgaaaagtgccacctgacgtcaggtaccaagcctaggcctccaaaaaagcctcctcactacttctggaatagctcagaggcagaggcggcctcggcctctgcataaataaaaaaaattagtcagccatggggcggagaatgggcggaactgggcggagttaggggcgggatgggcggagttaggggcgggactatggttgctgactaattgagatgcatgctttgcatacttctgcctgctggggagcctggggactttccacacctggttgctgactaattgagatgcatgctttgcatacttctgcctgctggggagcctggggactttccacaccggatccaccatggccaagttgaccagtgccgttccggtgctcaccgcgcgcgacgtcgccggagcggtcgagttctggaccgaccggctcgggttctcccgggacttcgtggaggacgacttcgccggtgtggtccgggacgacgtgaccctgttcatcagcgcggtccaggaccaggtggtgccggacaacaccctggcctgggtgtgggtgcgcggcctggacgagctgtacgccgagtggtcggaggtcgtgtccacgaacttccgggacgcctccgggccggccatgaccgagatcggcgagcagccgtgggggcgggagttcgccctgcgcgacccggccggcaactgcgtgcacttcgtggccgaggagcaggactgaacgcgtgctgtaagtctgcagaaattgatgatctattaaacaataaagatgtccactaaaatggaagtttttcctgtcatactttgttaagaagggtgagaacagagtacctacattttgaatggaaggattggagctacgggggtgggggtggggtgggattagataaatgcctgctctttactgaaggctctttactattgctttatgataatgtttcatagttggatatcataatttaaacaagcaaaaccaaattaagggccagctcattcctcccactcatgatctatggatctatagatctctcgtgcagctggggctctagggggtatccccacgcgccctgtagcggcgcattaagcgcggcgggtgtggtggttacgcgcagcgtgaccgctacacttgccagcgccctagcgcccgctcctttcgctttcttcccttcctttctcgccacgttcgccggctttccccgtcaagctctaaatcgggggctccctttagggttccgatttagtgctttacggcacctcgaccccaaaaaacttgattagggtgatggttcacgtagtgggccatcgccctgatagacggtttttcgccctttgacgttggagtccacgttctttaatagtggactcttgttccaaactggaacaacactcaaccctatctcggtctattcttttgatttataagggattttgccgatttcggcctattggttaaaaaatgagctgatttaacaaaaatttaacgcgaattaattctgtggaatgtgtgtcagttagtcgcgaggcctccgcgccgggttttggcgcctcccgcgggcgcccccctcctcacggcgagcgctgccacgtcagacgaagggcgcagcgagcgtcctgatccttccgcccggacgctcaggacagcggcccgctgctcataagactcggccttagaaccccagtatcagcagaaggacattttaggacgggacttgggtgactctagggcactggttttctttccagagagcggaacaggcgaggaaaagtagtcccttctcggcgattctgcggagggatctccgtggggcggtgaacgccgatgattatataaggacgcgccgggtgtggcacagctagttccgtcgcagccgggatttgggtcgcggttcttgtttgtggatcgctgtgatcgtcacttggtgagtagcgggctgctgggctggccggggctttcgtggccgccgggccgctcggtgggacggaagcgtgtggagagaccgccaagggctgtagtctgggtccgcgagcaaggttgccctgaactgggggttggggggagcgcagcaaaatggcggctgttcccgagtcttgaatggaagacgcttgtgaggcgggctgtgaggtcgttgaaacaaggtggggggcatggtgggcggcaagaacccaaggtcttgaggccttcgctaatgcgggaaagctcttattcgggtgagatgggctggggcaccatctggggaccctgacgtgaagtttgtcactgactggagaactcggtttgtcgtctgttgcgggggcggcagttatggcggtgccgttgggcagtgcacccgtacctttgggagcgcgcgccctcgtcgtgtcgtgacgtcacccgttctgttggcttataatgcagggtggggccacctgccggtaggtgtgcggtaggcttttctccgtcgcaggacgcagggttcgggcctagggtaggctctcctgaatcgacaggcgccggacctctggtgaggggagggataagtgaggcgtcagtttctttggtcggttttatgtacctatcttcttaagtagctgaagctccggttttgaactatgcgctcggggttggcgagtgtgttttgtgaagttttttaggcaccttttgaaatgtaatcatttgggtcaatatgtaattttcagtgttagactagtaaattgtccgctaaattctggccgtttttggcttttttgttagacgtcgaccgatcctgagaacttcagggtgagtttggggacccttgattgttctttctttttcgctattgtaaaattcatgttatatggagggggcaaagttttcagggtgttgtttagaatgggaagatgtcccttgtatcaccatggaccctcatgataattttgtttctttcactttctactctgttgacaaccattgtctcctcttattttcttttcattttctgtaactttttcgttaaactttagcttgcatttgtaacgaatttttaaattcacttttgtttatttgtcagattgtaagtactttctctaatcacttttttttcaaggcaatcagggtatattatattgtacttcagcacagttttagagaacaattgttataattaaatgataaggtagaatatttctgcatataaattctggctggcgtggaaatattcttattggtagaaacaactacaccctggtcatcatcctgcctttctctttatggttacaatgatatacactgtttgagatgaggataaaatactctgagtccaaaccgggcccctctgctaaccatgttcatgccttcttctctttcctacagctcctgggcaacgtgctggttgttgtgctgtctcatcattttggcaaagaatt

SEQ ID NO: 18 - DNA, 3264 bp, synthetic construct
  misc_feature 1..3264: note = Synthetic construct
  source 1..3264: mol_type = other DNA
ggcctccgcgccgggttttggcgcctcccgcgggcgcccccctcctcacggcgagcgctgccacgtcagacgaagggcgcagcgagcgtcctgatccttccgcccggacgctcaggacagcggcccgctgctcataagactcggccttagaaccccagtatcagcagaaggacattttaggacgggacttgggtgactctagggcactggttttctttccagagagcggaacaggcgaggaaaagtagtcccttctcggcgattctgcggagggatctccgtggggcggtgaacgccgatgattatataaggacgcgccgggtgtggcacagctagttccgtcgcagccgggatttgggtcgcggttcttgtttgtggatcgctgtgatcgtcacttggtgagtagcgggctgctgggctggccggggctttcgtggccgccgggccgctcggtgggacggaagcgtgtggagagaccgccaagggctgtagtctgggtccgcgagcaaggttgccctgaactgggggttggggggagcgcagcaaaatggcggctgttcccgagtcttgaatggaagacgcttgtgaggcgggctgtgaggtcgttgaaacaaggtggggggcatggtgggcggcaagaacccaaggtcttgaggccttcgctaatgcgggaaagctcttattcgggtgagatgggctggggcaccatctggggaccctgacgtgaagtttgtcactgactggagaactcggtttgtcgtctgttgcgggggcggcagttatggcggtgccgttgggcagtgcacccgtacctttgggagcgcgcgccctcgtcgtgtcgtgacgtcacccgttctgttggcttataatgcagggtggggccacctgccggtaggtgtgcggtaggcttttctccgtcgcaggacgcagggttcgggcctagggtaggctctcctgaatcgacaggcgccggacctctggtgaggggagggataagtgaggcgtcagtttctttggtcggttttatgtacctatcttcttaagtagctgaagctccggttttgaactatgcgctcggggttggcgagtgtgttttgtgaagttttttaggcaccttttgaaatgtaatcatttgggtcaatatgtaattttcagtgttagactagtaaattgtccgctaaattctggccgtttttggcttttttgttagacgtcgaccgatcctgagaacttcagggtgagtttggggacccttgattgttctttctttttcgctattgtaaaattcatgttatatggagggggcaaagttttcagggtgttgtttagaatgggaagatgtcccttgtatcaccatggaccctcatgataattttgtttctttcactttctactctgttgacaaccattgtctcctcttattttcttttcattttctgtaactttttcgttaaactttagcttgcatttgtaacgaatttttaaattcacttttgtttatttgtcagattgtaagtactttctctaatcacttttttttcaaggcaatcagggtatattatattgtacttcagcacagttttagagaacaattgttataattaaatgataaggtagaatatttctgcatataaattctggctggcgtggaaatattcttattggtagaaacaactacaccctggtcatcatcctgcctttctctttatggttacaatgatatacactgtttgagatgaggataaaatactctgagtccaaaccgggcccctctgctaaccatgttcatgccttcttctctttcctacagctcctgggcaacgtgctggttgttgtgctgtctcatcattttggcaaagaattaagcttatactcgagctctagattgggaacccgggtctctcgaattcatggtggtggtggctgctgctccttctgctgctacagctgctcctaaggtgctgctgctgtctggacagcctgcttctggaggaagagctctgcctctgatggtgcctggacctagagctgctggatctgaggcttctggaacacctcaggctagaaagagacagagactgacacatctgtctcctgaagaaaaggctctgagaagaaagctgaagaatagagtggctgctcagacagctagagatagaaagaaggctagaatgtctgaactggaacagcaggtggtggatctggaagaagaaaatcataagctgcagctggaaaatcagctgctgagagaaaagacacatggactggtggtggaaaatcaggaactgagaacaagactgggaatggatacactggatcctgatgaagtgcctgaagtggaagctaagggatctggagtgagactggtggctggatctgctgaatctgctgctggagctggacctgtggtgacatctcctgaacatctgcctatggattctgatacagtggcttcttctgattctgaatctgatatcctgctgggaatcctggataagctggatcctgtgatgttttttaagtgtccttctcctgaatctgcttctctggaagaactgcctgaagtgtatcctgaaggaccttcttctctgcctgcttctctgtctctgtctgtgggaacatcttctgctaagctggaagctatcaatgaactgatcagatttgatcatgtgtatacaaagcctctggtgctggaaatcccttctgaaacagaatctcagacaaatgtggtggtgaagatcgaagaagctcctctgtcttcttctgaagaagatcatcctgaatttatcgtgtctgtgaagaaggaacctctggaagatgattttatccctgaactgggaatctctaatctgctgtcttcttctcattgtctgagacctccttcttgtctgctggatgctcattctgattgtggatatgaaggatctccttctcctttttctgatatgtcttctcctctgggaacagatcattcttgggaagatacatttgctaatgaactgtttcctcagctgatctctgtgtgagcggccgctaatcagccataccacatttgtagaggttttacttgctttaaaaaacctcccacacctccccctgaacctgaaacataaaatgaatgcaattgttgttgttaacttgtttattgcagcttataatggttacaaataaagcaatagcatcacaaatttcacaaataaagcatttttttcactgcattctagttgtggtttgtccaaactcatcaatgtatcttatcatgtc

SEQ ID NO: 19 - protein, 447 aa, Homo sapiens
EVQVLESGGDLVQPGGSLRLSCAASGFTFSAYAMTWVRQAPGKGLEWVSAISGSGGSAYYADSVKGRFTISRDNSKNTVYLQMNSLRAEDTAVYYCAKDGAWKMSGLDVWGQGTTVIVSSASTKGPSVFPLAPCSRSTSESTAALGCLVKDYFPEPVTVSWNSGALTSGVHTFPAVLQSSGLYSLSSVVTVPSSSLGTKTYTCNVDHKPSNTKVDKRVESKYGPPCPPCPAPEFLGGPSVFLFPPKPKDTLMISRTPEVTCVVVDVSQEDPEVQFNWYVDGVEVHNAKTKPREEQFNSTYRVVSVLTVLHQDWLNGKEYKCKVSNKGLPSSIEKTISKAKGQPREPQVYTLPPSQEEMTKNQVSLTCLVKGFYPSDIAVEWESNGQPENNYKTTPPVLDSDGSFFLYSRLTVDKSRWQEGNVFSCSVMHEALHNHYTQKSLSLSLGK

SEQ ID NO: 20 - protein, 110 aa, Homo sapiens
ESGGDLVQPGGSLRLSCAASGFTFSAYAMTWVRQAPGKGLEWVSAISGSGGSAYYADSVKGRFTISRDNSKNTVYLQMNSLRAEDTAVYYCAKDGAWKMSGLDVWGQGTT

SEQ ID NO: 21 - protein, 214 aa, Homo sapiens
DIQMTQSPASLSASVGDRVTITCRASQDISDYLAWYQQKPGKIPRLLIYTTSTLQSGVPSRFRGSGSGTDFTLTISSLQPEDVATYYCQKYDSAPLTFGGGTKVEIKRTVAAPSVFIFPPSDEQLKSGTASVVCLLNNFYPREAKVQWKVDNALQSGNSQESVTEQDSKDSTYSLSSTLTLSKADYEKHKVYACEVTHQGLSSPVTKSFNRGEC

SEQ ID NO: 22 - protein, 100 aa, Homo sapiens
QSPASLSASVGDRVTITCRASQDISDYLAWYQQKPGKIPRLLIYTTSTLQSGVPSRFRGSGSGTDFTLTISSLQPEDVATYYCQKYDSAPLTFGGGTKVE

SEQ ID NO: 23 - DNA, 2971 bp, synthetic construct
  misc_feature 1..2971: note = Synthetic construct
  source 1..2971: mol_type = other DNA
tagttattaatagtaatcaattacggggtcattagttcatagcccatatatggagttccgcgttacataacttacggtaaatggcccgcctggctgaccgcccaacgacccccgcccattgacgtcaataatgacgtatgttcccatagtaacgccaatagggactttccattgacgtcaatgggtggagtatttacggtaaactgcccacttggcagtacatcaagtgtatcatatgccaagtacgccccctattgacgtcaatgacggtaaatggcccgcctggcattatgcccagtacatgaccttatgggactttcctacttggcagtacatctacgtattagtcatcgctattaccatggtgatgcggttttggcagtacatcaatgggcgtggatagcggtttgactcacggggatttccaagtctccaccccattgacgtcaatgggagtttgttttggcaccaaaatcaacgggactttccaaaatgtcgtaacaactccgccccattgacgcaaatgggcggtaggcgtgtacggtgggaggtctatataagcagagctcatgatagaagcactctactattcgtcgaccgatcctgagaacttcagggtgagtttggggacccttgattgttctttctttttcgctattgtaaaattcatgttatatggagggggcaaagttttcagggtgttgtttagaatgggaagatgtcccttgtatcaccatggaccctcatgataattttgtttctttcactttctactctgttgacaaccattgtctcctcttattttcttttcattttctgtaactttttcgttaaactttagcttgcatttgtaacgaatttttaaattcacttttgtttatttgtcagattgtaagtactttctctaatcacttttttttcaaggcaatcagggtatattatattgtacttcagcacagttttagagaacaattgttataattaaatgataaggtagaatatttctgcatataaattctggctggcgtggaaatattcttattggtagaaacaactacaccctggtcatcatcctgcctttctctttatggttacaatgatatacactgtttgagatgaggataaaatactctgagtccaaaccgggcccctctgctaaccatgttcatgccttcttctctttcctacagctcctgggcaacgtgctggttgttgtgctgtctcatcattttggcaaagaattaagcttatactcgagctctagattgggaacccgggtctctcgaattcgagatctccaccatgcacagacctagacgtcgtggaactcgtccacctccactggcactgctcgctgctctcctcctggctgcacgtggtgctgatgcagaggtgcaggtgttggagtctgggggagacttggtacagcctggggggtccctgagactctcctgtgcagcctctggattcacctttagtgcctatgccatgacctgggtccgccaggctccagggaaggggctggagtgggtctcagctattagtggtagtggtggtagcgcatactacgcagactccgtgaagggccggttcaccatctccagagacaattccaagaacacggtatatctgcagatgaacagcctgagagccgaggacacggccgtatattactgtgcgaaagatggggcctggaaaatgtccggtttggacgtctggggccaagggaccacggtcatcgtctcctcagcctccaccaagggcccatcggtcttccccctggcgccctgctccaggagcacctccgagagcacagccgccctgggctgcctggtcaaggactacttccccgaaccggtgacggtgtcgtggaactcaggcgccctgaccagcggcgtgcacaccttcccggctgtcctacagtcctcaggactctactccctcagcagcgtggtgaccgtgccctccagcagcttgggcacgaagacctacacctgcaacgtagatcacaagcccagcaacaccaaggtggacaagagagttgagtccaaatatggtcccccatgcccaccctgcccagcacctgagttcctggggggaccatcagtcttcctgttccccccaaaacccaaggacactctcatgatctcccggacccctgaggtcacgtgcgtggtggtggacgtgagccaggaagaccccgaggtccagttcaactggtacgtggatggcgtggaggtgcataatgccaagacaaagccgcgggaggagcagttcaacagcacgtaccgtgtggtcagcgtcctcaccgtcctgcaccaggactggctgaacggcaaggagtacaagtgcaaggtctccaacaaaggcctcccgtcctccatcgagaaaaccatctccaaagccaaagggcagccccgagagccacaggtgtacaccctgcccccatcccaggaggagatgaccaagaaccaggtcagcctgacctgcctggtcaaaggcttctaccccagcgacatcgccgtggagtgggagagcaatgggcagccggagaacaactacaagaccacgcctcccgtgctggactccgacggctccttcttcctctacagcaggctcaccgtggacaagagcaggtggcaggaggggaatgtcttctcatgctccgtgatgcatgaggctctgcacaaccactacacacagaagtccctctccctgtctctgggtaaatgagcggccgctaatcagccataccacatttgtagaggttttacttgctttaaaaaacctcccacacctccccctgaacctgaaacataaaatgaatgcaattgttgttgttaacttgtttattgcagcttataatggttacaaataaagcaatagcatcacaaatttcacaaataaagcatttttttcactgcattctagttgtggtttgtccaaactcatcaatgtatcttatcatgtc

SEQ ID NO: 24 - DNA, 7013 bp, synthetic construct
  misc_feature 1..7013: note = Synthetic plasmid
  source 1..7013: mol_type = other DNA
tcgcgatgtgtgactagttagttattaatagtaatcaattacggggtcattagttcatagcccatatatggagttccgcgttacataacttacggtaaatggcccgcctggctgaccgcccaacgacccccgcccattgacgtcaataatgacgtatgttcccatagtaacgccaatagggactttccattgacgtcaatgggtggagtatttacggtaaactgcccacttggcagtacatcaagtgtatcatatgccaagtacgccccctattgacgtcaatgacggtaaatggcccgcctggcattatgcccagtacatgaccttatgggactttcctacttggcagtacatctacgtattagtcatcgctattaccatggtgatgcggttttggcagtacatcaatgggcgtggatagcggtttgactcacggggatttccaagtctccaccccattgacgtcaatgggagtttgttttggcaccaaaatcaacgggactttccaaaatgtcgtaacaactccgccccattgacgcaaatgggcggtaggcgtgtacggtgggaggtctatataagcagagctcatgatagaagcactctactattcgtcgaccgatcctgagaacttcagggtgagtttggggacccttgattgttctttctttttcgctattgtaaaattcatgttatatggagggggcaaagttttcagggtgttgtttagaatgggaagatgtcccttgtatcaccatggaccctcatgataattttgtttctttcactttctactctgttgacaaccattgtctcctcttattttcttttcattttctgtaactttttcgttaaactttagcttgcatttgtaacgaatttttaaattcacttttgtttatttgtcagattgtaagtactttctctaatcacttttttttcaaggcaatcagggtatattatattgtacttcagcacagttttagagaacaattgttataattaaatgataaggtagaatatttctgcatataaattctggctggcgtggaaatattcttattggtagaaacaactacaccctggtcatcatcctgcctttctctttatggttacaatgatatacactgtttgagatgaggataaaatactctgagtccaaaccgggcccctctgctaaccatgttcatgccttcttctctttcctacagctcctgggcaacgtgctggttgttgtgctgtctcatcattttggcaaagaattaagcttatactcgagctctagattgggaacccgggtctctcgaattcgagatctccaccatgcacagacctagacgtcgtggaactcgtccacctccactggcactgctcgctgctctcctcctggctgcacgtggtgctgatgcagaggtgcaggtgttggagtctgggggagacttggtacagcctggggggtccctgagactctcctgtgcagcctctggattcacctttagtgcctatgccatgacctgggtccgccaggctccagggaaggggctggagtgggtctcagctattagtggtagtggtggtagcgcatactacgcagactccgtgaagggccggttcaccatctccagagacaattccaagaacacggtatatctgcagatgaacagcctgagagccgaggacacggccgtatattactgtgcgaaagatggggcctggaaaatgtccggtttggacgtctggggccaagggaccacggtcatcgtctcctcagcctccaccaagggcccatcggtcttccccctggcgccctgctccaggagcacctccgagagcacagccgccctgggctgcctggtcaaggactacttccccgaaccggtgacggtgtcgtggaactcaggcgccctgaccagcggcgtgcacaccttcccggctgtcctacagtcctcaggactctactccctcagcagcgtggtgaccgtgccctccagcagcttgggcacgaagacctacacctgcaacgtagatcacaagcccagcaacaccaaggtggacaagagagttgagtccaaatatggtcccccatgcccaccctgcccagcacctgagttcctggggggaccatcagtcttcctgttccccccaaaacccaaggacactctcatgatctcccggacccctgaggtcacgtgcgtggtggtggacgtgagccaggaagaccccgaggtccagttcaactggtacgtggatggcgtggaggtgcataatgccaagacaaagccgcgggaggagcagttcaacagcacgtaccgtgtggtcagcgtcctcaccgtcctgcaccaggactggctgaacggcaaggagtacaagtgcaaggtctccaacaaaggcctcccgtcctccatcgagaaaaccatctccaaagccaaagggcagccccgagagccacaggtgtacaccctgcccccatcccaggaggagatgaccaagaaccaggtcagcctgacctgcctggtcaaaggcttctaccccagcgacatcgccgtggagtgggagagcaatgggcagccggagaacaactacaagaccacgcctcccgtgctggactccgacggctccttcttcctctacagcaggctcaccgtggacaagagcaggtggcaggaggggaatgtcttctcatgctccgtgatgcatgaggctctgcacaaccactacacacagaagtccctctccctgtctctgggtaaatgagcggccgctaatcagccataccacatttgtagaggttttacttgctttaaaaaacctcccacacctccccctgaacctgaaacataaaatgaatgcaattgttgttgttaacttgtttattgcagcttataatggttacaaataaagcaatagcatcacaaatttcacaaataaagcatttttttcactgcattctagttgtggtttgtccaaactcatcaatgtatcttatcatgtctaccggtcctgcagggcccctctcttcatgtgagcaaaaggccagcaaaaggccaggaaccgtaaaaaggccgcgttgctggcgtttttccataggctccgcccccctgacgagcatcacaaaaatcgacgctcaagtcagaggtggcgaaacccgacaggactataaagataccaggcgtttccccctggaagctccctcgtgcgctctcctgttccgaccctgccgcttaccggatacctgtccgcctttctcccttcgggaagcgtggcgctttctcaatgctcacgctgtaggtatctcagttcggtgtaggtcgttcgctccaagctgggctgtgtgcacgaaccccccgttcagcccgaccgctgcgccttatccggtaactatcgtcttgagtccaacccggtaagacacgacttatcgccactggcagcagccactggtaacaggattagcagagcgaggtatgtaggcggtgctacagagttcttgaagtggtggcctaactacggctacactagaaggacagtatttggtatctgcgctctgctgaagccagttaccttcggaaaaagagttggtagctcttgatccggcaaacaaaccaccgctggtagcggtggtttttttgtttgcaagcagcagattacgcgcagaaaaaaaggatctcaagaagatcctttgatcttttctacggggtctgacgctcagtggaacgaaaactcacgttaagggattttggtcatgggcgcgcctcatactcctgcaggcatgagattatcaaaaaggatcttcacctagatccttttaaattaaaaatgaagttttaaatcaatctaaagtatatatgagtaaacttggtctgacagttaccaatgcttaatcagtgaggcacctatctcagcgatctgtctatttcgttcatccatagttgcctgactccccgtcgtgtagataactacgatacgggagggcttaccatctggccccagtgctgcaatgataccgcgagacccacgctcaccggctccagatttatcagcaataaaccagccagccggaagggccgagcgcagaagtggtcctgcaactttatccgcctccatccagtctattaattgttgccgggaagctagagtaagtagttcgccagttaatagtttgcgcaacgttgttgccattgctacaggcatcgtggtgtcacgctcgtcgtttggtatggcttcattcagctccggttcccaacgatcaaggcgagttacatgatcccccatgttgtgcaaaaaagcggttagctccttcggtcctccgatcgttgtcagaagtaagttggccgcagtgttatcactcatggttatggcagcactgcataattctcttactgtcatgccatccgtaagatgcttttctgtgactggtgagtactcaaccaagtcattctgagaatagtgtatgcggcgaccgagttgctcttgcccggcgtcaatacgggataataccgcgccacatagcagaactttaaaagtgctcatcattggaaaacgttcttcggggcgaaaactctcaaggatcttaccgctgttgagatccagttcgatgtaacccactcgtgcacccaactgatcttcagcatcttttactttcaccagcgtttctgggtgagcaaaaacaggaaggcaaaatgccgcaaaaaagggaataagggcgacacggaaatgttgaatactcatactcttcctttttcaatattattgaagcatttatcagggttattgtctcatgagcggatacatatttgaatgtatttagaaaaataaacaaataggggttccgcgcacatttccccgaaaagtgccacctgacgtcaggtaccaagcctaggcctccaaaaaagcctcctcactacttctggaatagctcagaggcagaggcggcctcggcctctgcataaataaaaaaaattagtcagccatggggcggagaatgggcggaactgggcggagttaggggcgggatgggcggagttaggggcgggactatggttgctgactaattgagatgcatgctttgcatacttctgcctgctggggagcctggggactttccacacctggttgctgactaattgagatgcatgctttgcatacttctgcctgctggggagcctggggactttccacaccggatccaccatggatagatccggaaagcctgaactcaccgcgacgtctgtcgagaagtttctgatcgaaaagttcgacagcgtctccgacctgatgcagctctcggagggcgaagaatctcgtgctttcagcttcgatgtaggagggcgtggatatgtcctgcgggtaaatagctgcgccgatggtttctacaaagatcgttatgtttatcggcactttgcatcggccgcgctcccgattccggaagtgcttgacattggggagttcagcgagagcctgacctattgcatctcccgccgtgcacagggtgtcacgttgcaagacctgcctgaaaccgaactgcccgctgttctgcagccggtcgcggaggccatggatgcgatcgctgcggccgatcttagccagacgagcgggttcggcccattcggaccgcaaggaatcggtcaatacactacatggcgtgatttcatatgcgcgattgctgatccccatgtgtatcactggcaaactgtgatggacgacaccgtcagtgcgtccgtcgcgcaggctctcgatgagctgatgctttgggccgaggactgccccgaagtccggcacctcgtgcacgcggatttcggctccaacaatgtcctgacggacaatggccgcataacagcggtcattgactggagcgaggcgatgttcggggattcccaatacgaggtcgccaacatcttcttctggaggccgtggttggcttgtatggagcagcagacgcgctacttcgagcggaggcatccggagcttgcaggatcgccgcggctccgggcgtatatgctccgcattggtcttgaccaactctatcagagcttggttgacggcaatttcgatgatgcagcttgggcgcagggtcgatgcgacgcaatcgtccgatccggagccgggactgtcgggcgtacacaaatcgcccgcagaagcgcggccgtctggaccgatggctgtgtagaagtactcgccgatagtggaaaccgacgccccagcactcgtccgagggcaaaggaatagacgcgtgctgtaagtctgcagaaattgatgatctattaaacaataaagatgtccactaaaatggaagtttttcctgtcatactttgttaagaagggtgagaacagagtacctacattttgaatggaaggattggagctacgggggtgggggtggggtgggattagataaatgcctgctctttactgaaggctctttactattgctttatgataatgtttcatagttggatatcataatttaaacaagcaaaaccaaattaagggccagctcattcctcccactcatgatctatggatctatagatctctcgtgcagctggggctctagggggtatccccacgcgccctgtagcggcgcattaagcgcggcgggtgtggtggttacgcgcagcgtgaccgctacacttgccagcgccctagcgcccgctcctttcgctttcttcccttcctttctcgccacgttcgccggctttccccgtcaagctctaaatcgggggctccctttagggttccgatttagtgctttacggcacctcgaccccaaaaaacttgattagggtgatggttcacgtagtgggccatcgccctgatagacggtttttcgccctttgacgttggagtccacgttctttaatagtggactcttgttccaaactggaacaacactcaaccctatctcggtctattcttttgatttataagggattttgccgatttcggcctattggttaaaaaatgagctgatttaacaaaaatttaacgcgaattaattctgtggaatgtgtgtcagttag

SEQ ID NO: 25 - DNA, 2272 bp, synthetic construct
  misc_feature 1..2272: note = Synthetic construct
  source 1..2272: mol_type = other DNA
tagttattaatagtaatcaattacggggtcattagttcatagcccatatatggagttccgcgttacataacttacggtaaatggcccgcctggctgaccgcccaacgacccccgcccattgacgtcaataatgacgtatgttcccatagtaacgccaatagggactttccattgacgtcaatgggtggagtatttacggtaaactgcccacttggcagtacatcaagtgtatcatatgccaagtacgccccctattgacgtcaatgacggtaaatggcccgcctggcattatgcccagtacatgaccttatgggactttcctacttggcagtacatctacgtattagtcatcgctattaccatggtgatgcggttttggcagtacatcaatgggcgtggatagcggtttgactcacggggatttccaagtctccaccccattgacgtcaatgggagtttgttttggcaccaaaatcaacgggactttccaaaatgtcgtaacaactccgccccattgacgcaaatgggcggtaggcgtgtacggtgggaggtctatataagcagagctcatgatagaagcactctactattcgtcgaccgatcctgagaacttcagggtgagtttggggacccttgattgttctttctttttcgctattgtaaaattcatgttatatggagggggcaaagttttcagggtgttgtttagaatgggaagatgtcccttgtatcaccatggaccctcatgataattttgtttctttcactttctactctgttgacaaccattgtctcctcttattttcttttcattttctgtaactttttcgttaaactttagcttgcatttgtaacgaatttttaaattcacttttgtttatttgtcagattgtaagtactttctctaatcacttttttttcaaggcaatcagggtatattatattgtacttcagcacagttttagagaacaattgttataattaaatgataaggtagaatatttctgcatataaattctggctggcgtggaaatattcttattggtagaaacaactacaccctggtcatcatcctgcctttctctttatggttacaatgatatacactgtttgagatgaggataaaatactctgagtccaaaccgggcccctctgctaaccatgttcatgccttcttctctttcctacagctcctgggcaacgtgctggttgttgtgctgtctcatcattttggcaaagaattaagcttatactcgagctctagattgggaacccgggtctctcgaattcgagatctccaccatgcacagacctagacgtcgtggaactcgtccacctccactggcactgctcgctgctctcctcctggctgcacgtggtgctgatgcagacatccagatgacccagtctccagcctccctgtctgcatctgttggagacagagtcaccatcacttgtcgggcgagtcaggacattagcgattatttagcctggtatcagcagaaaccagggaaaattcctaggctcctgatctatactacatccactttgcaatcaggggtcccatctcggttccgtggcagtgggtctgggacagatttcactctcaccatcagcagcctgcagcctgaagatgttgcaacttattactgtcagaagtatgacagtgccccgctcactttcggcggagggaccaaggtggagatcaaacgaactgtggctgcaccatctgtcttcatcttcccgccatctgatgagcagttgaaatctggaactgcctctgttgtgtgcctgctgaataacttctatcccagagaggccaaagtacagtggaaggtggataacgccctccaatcgggtaactcccaggagagtgtcacagagcaggacagcaaggacagcacctacagcctcagcagcaccctgacgctgagcaaagcagactacgagaaacacaaagtctacgcctgcgaagtcacccatcagggcctgagctcgcccgtcacaaagagcttcaacaggggagagtgttaggcggccgctaatcagccataccacatttgtagaggttttacttgctttaaaaaacctcccacacctccccctgaacctgaaacataaaatgaatgcaattgttgttgttaacttgtttattgcagcttataatggttacaaataaagcaatagcatcacaaatttcacaaataaagcatttttttcactgcattctagttgtggtttgtccaaactcatcaatgtatcttatcatgtc

SEQ ID NO: 26 - DNA, 6335 bp, synthetic construct
  misc_feature 1..6335: note = Synthetic plasmid
  source 1..6335: mol_type = other DNA
tcgagctctagattgggaacccgggtctctcgaattcgagatctccaccatgcacagacctagacgtcgtggaactcgtccacctccactggcactgctcgctgctctcctcctggctgcacgtggtgctgatgcagacatccagatgacccagtctccagcctccctgtctgcatctgttggagacagagtcaccatcacttgtcgggcgagtcaggacattagcgattatttagcctggtatcagcagaaaccagggaaaattcctaggctcctgatctatactacatccactttgcaatcaggggtcccatctcggttccgtggcagtgggtctgggacagatttcactctcaccatcagcagcctgcagcctgaagatgttgcaacttattactgtcagaagtatgacagtgccccgctcactttcggcggagggaccaaggtggagatcaaacgaactgtggctgcaccatctgtcttcatcttcccgccatctgatgagcagttgaaatctggaactgcctctgttgtgtgcctgctgaataacttctatcccagagaggccaaagtacagtggaaggtggataacgccctccaatcgggtaactcccaggagagtgtcacagagcaggacagcaaggacagcacctacagcctcagcagcaccctgacgctgagcaaagcagactacgagaaacacaaagtctacgcctgcgaagtcacccatcagggcctgagctcgcccgtcacaaagagcttcaacaggggagagtgttaggcggccgctaatcagccataccacatttgtagaggttttacttgctttaaaaaacctcccacacctccccctgaacctgaaacataaaatgaatgcaattgttgttgttaacttgtttattgcagcttataatggttacaaataaagcaatagcatcacaaatttcacaaataaagcatttttttcactgcattctagttgtggtttgtccaaactcatcaatgtatcttatcatgtctaccggtagggcccctctcttcatgtgagcaaaaggccagcaaaaggccaggaaccgtaaaaaggccgcgttgctggcgtttttccataggctccgcccccctgacgagcatcacaaaaatcgacgctcaagtcagaggtggcgaaacccgacaggactataaagataccaggcgtttccccctggaagctccctcgtgcgctctcctgttccgaccctgccgcttaccggatacctgtccgcctttctcccttcgggaagcgtggcgctttctcaatgctcacgctgtaggtatctcagttcggtgtaggtcgttcgctccaagctgggctgtgtgcacgaaccccccgttcagcccgaccgctgcgccttatccggtaactatcgtcttgagtccaacccggtaagacacgacttatcgccactggcagcagccactggtaacaggattagcagagcgaggtatgtaggcggtgctacagagttcttgaagtggtggcctaactacggctacactagaaggacagtatttggtatctgcgctctgctgaagccagttaccttcggaaaaagagttggtagctcttgatccggcaaacaaaccaccgctggtagcggtggtttttttgtttgcaagcagcagattacgcgcagaaaaaaaggatctcaagaagatcctttgatcttttctacggggtctgacgctcagtggaacgaaaactcacgttaagggattttggtcatgggcgcgggcatgagattatcaaaaaggatcttcacctagatccttttaaattaaaaatgaagttttaaatcaatctaaagtatatatgagtaaacttggtctgacagttaccaatgcttaatcagtgaggcacctatctcagcgatctgtctatttcgttcatccatagttgcctgactccccgtcgtgtagataactacgatacgggagggcttaccatctggccccagtgctgcaatgataccgcgagacccacgctcaccggctccagatttatcagcaataaaccagccagccggaagggccgagcgcagaagtggtcctgcaactttatccgcctccatccagtctattaattgttgccgggaagctagagtaagtagttcgccagttaatagtttgcgcaacgttgttgccattgctacaggcatcgtggtgtcacgctcgtcgtttggtatggcttcattcagctccggttcccaacgatcaaggcgagttacatgatcccccatgttgtgcaaaaaagcggttagctccttcggtcctccgatcgttgtcagaagtaagttggccgcagtgttatcactcatggttatggcagcactgcataattctcttactgtcatgccatccgtaagatgcttttctgtgactggtgagtactcaaccaagtcattctgagaatagtgtatgcggcgaccgagttgctcttgcccggcgtcaatacgggataataccgcgccacatagcagaactttaaaagtgctcatcattggaaaacgttcttcggggcgaaaactctcaaggatcttaccgctgttgagatccagttcgatgtaacccactcgtgcacccaactgatcttcagcatcttttactttcaccagcgtttctgggtgagcaaaaacaggaaggcaaaatgccgcaaaaaagggaataagggcgacacggaaatgttgaatactcatactcttcctttttcaatattattgaagcatttatcagggttattgtctcatgagcggatacatatttgaatgtatttagaaaaataaacaaataggggttccgcgcacatttccccgaaaagtgccacctgacgtcaggtacacttaggcgcgccattagagttcctgcaggctacatggtaccaagcctaggcctccaaaaaagcctcctcactacttctggaatagctcagaggcagaggcggcctcggcctctgcataaataaaaaaaattagtcagccatggggcggagaatgggcggaactgggcggagttaggggcgggatgggcggagttaggggcgggactatggttgctgactaattgagatgcatgctttgcatacttctgcctgctggggagcctggggactttccacacctggttgctgactaattgagatgcatgctttgcatacttctgcctgctggggagcctggggactttccacaccggatccaccatggatagatccggaaagcctgaactcaccgcgacgtctgtcgagaagtttctgatcgaaaagttcgacagcgtctccgacctgatgcagctctcggagggcgaagaatctcgtgctttcagcttcgatgtaggagggcgtggatatgtcctgcgggtaaatagctgcgccgatggtttctacaaagatcgttatgtttatcggcactttgcatcggccgcgctcccgattccggaagtgcttgacattggggagttcagcgagagcctgacctattgcatctcccgccgtgcacagggtgtcacgttgcaagacctgcctgaaaccgaactgcccgctgttctgcagccggtcgcggaggccatggatgcgatcgctgcggccgatcttagccagacgagcgggttcggcccattcggaccgcaaggaatcggtcaatacactacatggcgtgatttcatatgcgcgattgctgatccccatgtgtatcactggcaaactgtgatggacgacaccgtcagtgcgtccgtcgcgcaggctctcgatgagctgatgctttgggccgaggactgccccgaagtccggcacctcgtgcacgcggatttcggctccaacaatgtcctgacggacaatggccgcataacagcggtcattgactggagcgaggcgatgttcggggattcccaatacgaggtcgccaacatcttcttctggaggccgtggttggcttgtatggagcagcagacgcgctacttcgagcggaggcatccggagcttgcaggatcgccgcggctccgggcgtatatgctccgcattggtcttgaccaactctatcagagcttggttgacggcaatttcgatgatgcagcttgggcgcagggtcgatgcgacgcaatcgtccgatccggagccgggactgtcgggcgtacacaaatcgcccgcagaagcgcggccgtctggaccgatggctgtgtagaagtactcgccgatagtggaaaccgacgccccagcactcgtccgagggcaaaggaatagacgcgtgctgtaagtctgcagaaattgatgatctattaaacaataaagatgtccactaaaatggaagtttttcctgtcatactttgttaagaagggtgagaacagagtacctacattttgaatggaaggattggagctacgggggtgggggtggggtgggattagataaatgcctgctctttactgaaggctctttactattgctttatgataatgtttcatagttggatatcataatttaaacaagcaaaaccaaattaagggccagctcattcctcccactcatgatctatggatctatagatctctcgtgcagctggggctctagggggtatccccacgcgccctgtagcggcgcattaagcgcggcgggtgtggtggttacgcgcagcgtgaccgctacacttgccagcgccctagcgcccgctcctttcgctttcttcccttcctttctcgccacgttcgccggctttccccgtcaagctctaaatcgggggctccctttagggttccgatttagtgctttacggcacctcgaccccaaaaaacttgattagggtgatggttcacgtagtgggccatcgccctgatagacggtttttcgccctttgacgttggagtccacgttctttaatagtggactcttgttccaaactggaacaacactcaaccctatctcggtctattcttttgatttataagggattttgccgatttcggcctattggttaaaaaatgagctgatttaacaaaaatttaacgcgaattaattctgtggaatgtgtgtcagttagtcgcgatgtgtgactagttagttattaatagtaatcaattacggggtcattagttcatagcccatatatggagttccgcgttacataacttacggtaaatggcccgcctggctgaccgcccaacgacccccgcccattgacgtcaataatgacgtatgttcccatagtaacgccaatagggactttccattgacgtcaatgggtggagtatttacggtaaactgcccacttggcagtacatcaagtgtatcatatgccaagtacgccccctattgacgtcaatgacggtaaatggcccgcctggcattatgcccagtacatgaccttatgggactttcctacttggcagtacatctacgtattagtcatcgctattaccatggtgatgcggttttggcagtacatcaatgggcgtggatagcggtttgactcacggggatttccaagtctccaccccattgacgtcaatgggagtttgttttggcaccaaaatcaacgggactttccaaaatgtcgtaacaactccgccccattgacgcaaatgggcggtaggcgtgtacggtgggaggtctatataagcagagctcatgatagaagcactctactattcgtcgaccgatcctgagaacttcagggtgagtttggggacccttgattgttctttctttttcgctattgtaaaattcatgttatatggagggggcaaagttttcagggtgttgtttagaatgggaagatgtcccttgtatcaccatggaccctcatgataattttgtttctttcactttctactctgttgacaaccattgtctcctcttattttcttttcattttctgtaactttttcgttaaactttagcttgcatttgtaacgaatttttaaattcacttttgtttatttgtcagattgtaagtactttctctaatcacttttttttcaaggcaatcagggtatattatattgtacttcagcacagttttagagaacaattgttataattaaatgataaggtagaatatttctgcatataaattctggctggcgtggaaatattcttattggtagaaacaactacaccctggtcatcatcctgcctttctctttatggttacaatgatatacactgtttgagatgaggataaaatactctgagtccaaaccgggcccctctgctaaccatgttcatgccttcttctctttcctacagctcctgggcaacgtgctggttgttgtgctgtctcatcattttggcaaagaattaagcttatac

SEQ ID NO: 27 - protein, 452 aa, Homo sapiens
EVQLVESGGGLVQPGGSLRLSCAASGFTFSSYDIHWVRQATGKGLEWVSAIGPAGDTYYPGSVKGRFTISRENAKNSLYLQMNSLRAGDTAVYYCARGLITFGGLIAPFDYWGQGTLVTVSSASTKGPSVFPLAPSSKSTSGGTAALGCLVKDYFPEPVTVSWNSGALTSGVHTFPAVLQSSGLYSLSSVVTVPSSSLGTQTYICNVNHKPSNTKVDKKVEPKSCDKTHTCPPCPAPELLGGPSVFLFPPKPKDTLMISRTPEVTCVVVDVSHEDPEVKFNWYVDGVEVHNAKTKPREEQYNSTYRVVSVLTVLHQDWLNGKEYKCKVSNKALPAPIEKTISKAKGQPREPQVYTLPPSRDELTKNQVSLTCLVKGFYPSDIAVEWESNGQPENNYKTTPPVLDSDGSFFLYSKLTVDKSRWQQGNVFSCSVMHEALHNHYTQKSLSLSPGK

SEQ ID NO: 28 - protein, 112 aa, Homo sapiens
ESGGGLVQPGGSLRLSCAASGFTFSSYDIHWVRQATGKGLEWVSAIGPAGDTYYPGSVKGRFTISRENAKNSLYLQMNSLRAGDTAVYYCARGLITFGGLIAPFDYWGQGTL

SEQ ID NO: 29 - protein, 214 aa, Homo sapiens
EIVLTQSPGTLSLSPGERATLSCRASQSVSSTYLAWYQQKPGQAPRLLIYGASSRATGIPDRFSGSGSGTDFTLTISRLEPEDFAVYYCQHYDNSQTFGQGTKVEIKRTVAAPSVFIFPPSDEQLKSGTASVVCLLNNFYPREAKVQWKVDNALQSGNSQESVTEQDSKDSTYSLSSTLTLSKADYEKHKVYACEVTHQGLSSPVTKSFNRGEC

SEQ ID NO: 30 - protein, 107 aa, Homo sapiens
IVLTQSPGTLSLSPGERATLSCRASQSVSSTYLAWYQQKPGQAPRLLIYGASSRATGIPDRFSGSGSGTDFTLTISRLEPEDFAVYYCQHYDNSQTFGQGTKVEIKR

SEQ ID NO: 31 - DNA, 2986 bp, synthetic construct
  misc_feature 1..2986: note = Synthetic construct
  source 1..2986: mol_type = other DNA
tagttattaatagtaatcaattacggggtcattagttcatagcccatatatggagttccgcgttacataacttacggtaaatggcccgcctggctgaccgcccaacgacccccgcccattgacgtcaataatgacgtatgttcccatagtaacgccaatagggactttccattgacgtcaatgggtggagtatttacggtaaactgcccacttggcagtacatcaagtgtatcatatgccaagtacgccccctattgacgtcaatgacggtaaatggcccgcctggcattatgcccagtacatgaccttatgggactttcctacttggcagtacatctacgtattagtcatcgctattaccatggtgatgcggttttggcagtacatcaatgggcgtggatagcggtttgactcacggggatttccaagtctccaccccattgacgtcaatgggagtttgttttggcaccaaaatcaacgggactttccaaaatgtcgtaacaactccgccccattgacgcaaatgggcggtaggcgtgtacggtgggaggtctatataagcagagctcatgatagaagcactctactattcgtcgaccgatcctgagaacttcagggtgagtttggggacccttgattgttctttctttttcgctattgtaaaattcatgttatatggagggggcaaagttttcagggtgttgtttagaatgggaagatgtcccttgtatcaccatggaccctcatgataattttgtttctttcactttctactctgttgacaaccattgtctcctcttattttcttttcattttctgtaactttttcgttaaactttagcttgcatttgtaacgaatttttaaattcacttttgtttatttgtcagattgtaagtactttctctaatcacttttttttcaaggcaatcagggtatattatattgtacttcagcacagttttagagaacaattgttataattaaatgataaggtagaatatttctgcatataaattctggctggcgtggaaatattcttattggtagaaacaactacaccctggtcatcatcctgcctttctctttatggttacaatgatatacactgtttgagatgaggataaaatactctgagtccaaaccgggcccctctgctaaccatgttcatgccttcttctctttcctacagctcctgggcaacgtgctggttgttgtgctgtctcatcattttggcaaagaattaagcttatactcgagctctagattgggaacccgggtctctcgaattcgagatctccaccatgcacagacctagacgtcgtggaactcgtccacctccactggcactgctcgctgctctcctcctggctgcacgtggtgctgatgcagaggtgcagctggtggagtctgggggaggcttggtacagccgggggggtccctgagactctcctgtgcagcctctggattcaccttcagtagctacgacatacactgggtccgtcaagctacaggaaaaggtctggagtgggtctcagctattggtcctgctggtgacacatactatccaggctccgtgaagggccgattcaccatctccagagaaaatgccaagaactccttgtatcttcaaatgaacagcctgagagccggggacacggctgtgtattactgtgcaagaggtttgattacgtttggggggcttatcgccccgtttgactactggggccagggaaccctggtcaccgtctcctcagcctccaccaagggcccatcggtcttccccctggcaccctcctccaagagcacctctgggggcacagcggccctgggctgcctggtcaaggactacttccccgaaccggtgacggtgtcgtggaactcaggcgccctgaccagcggcgtgcacaccttcccggctgtcctacagtcctcaggactctactccctcagcagcgtggtgaccgtgccctccagcagcttgggcacccagacctacatctgcaacgtgaatcacaagcccagcaacaccaaggtggacaagaaagttgagcccaaatcttgtgacaaaactcacacatgcccaccgtgcccagcacctgaactcctggggggaccgtcagtcttcctcttccccccaaaacccaaggacaccctcatgatctcccggacccctgaggtcacatgcgtggtggtggacgtgagccacgaagaccctgaggtcaagttcaactggtacgtggacggcgtggaggtgcataatgccaagacaaagccgcgggaggagcagtacaacagcacgtaccgtgtggtcagcgtcctcaccgtcctgcaccaggactggctgaatggcaaggagtacaagtgcaaggtctccaacaaagccctcccagcccccatcgagaaaaccatctccaaagccaaagggcagccccgagaaccacaggtgtacaccctgcccccatcccgggatgagctgaccaagaaccaggtcagcctgacctgcctggtcaaaggcttctatcccagcgacatcgccgtggagtgggagagcaatgggcagccggagaacaactacaagaccacgcctcccgtgctggactccgacggctccttcttcctctacagcaagctcaccgtggacaagagcaggtggcagcaggggaacgtcttctcatgctccgtgatgcatgaggctctgcacaaccactacacgcagaagtccctctccctgtctccgggtaaatgagcggccgctaatcagccataccacatttgtagaggttttacttgctttaaaaaacctcccacacctccccctgaacctgaaacataaaatgaatgcaattgttgttgttaacttgtttattgcagcttataatggttacaaataaagcaatagcatcacaaatttcacaaataaagcatttttttcactgcattctagttgtggtttgtccaaactcatcaatgtatcttatcatgtc

SEQ ID NO: 32 - DNA, 7028 bp, synthetic construct
  misc_feature 1..7028: note = Synthetic plasmid
  source 1..7028: mol_type = other DNA
tcgcgatgtgtgactagttagttattaatagtaatcaattacggggtcattagttcatagcccatatatggagttccgcgttacataacttacggtaaatggcccgcctggctgaccgcccaacgacccccgcccattgacgtcaataatgacgtatgttcccatagtaacgccaatagggactttccattgacgtcaatgggtggagtatttacggtaaactgcccacttggcagtacatcaagtgtatcatatgccaagtacgccccctattgacgtcaatgacggtaaatggcccgcctggcattatgcccagtacatgaccttatgggactttcctacttggcagtacatctacgtattagtcatcgctattaccatggtgatgcggttttggcagtacatcaatgggcgtggatagcggtttgactcacggggatttccaagtctccaccccattgacgtcaatgggagtttgttttggcaccaaaatcaacgggactttccaaaatgtcgtaacaactccgccccattgacgcaaatgggcggtaggcgtgtacggtgggaggtctatataagcagagctcatgatagaagcactctactattcgtcgaccgatcctgagaacttcagggtgagtttggggacccttgattgttctttctttttcgctattgtaaaattcatgttatatggagggggcaaagttttcagggtgttgtttagaatgggaagatgtcccttgtatcaccatggaccctcatgataattttgtttctttcactttctactctgttgacaaccattgtctcctcttattttcttttcattttctgtaactttttcgttaaactttagcttgcatttgtaacgaatttttaaattcacttttgtttatttgtcagattgtaagtactttctctaatcacttttttttcaaggcaatcagggtatattatattgtacttcagcacagttttagagaacaattgttataattaaatgataaggtagaatatttctgcatataaattctggctggcgtggaaatattcttattggtagaaacaactacaccctggtcatcatcctgcctttctctttatggttacaatgatatacactgtttgagatgaggataaaatactctgagtccaaaccgggcccctctgctaaccatgttcatgccttcttctctttcctacagctcctgggcaacgtgctggttgttgtgctgtctcatcattttggcaaagaattaagcttatactcgagctctagattgggaacccgggtctctcgaattcgagatctccaccatgcacagacctagacgtcgtggaactcgtccacctccactggcactgctcgctgctctcctcctggctgcacgtggtgctgatgcagaggtgcagctggtggagtctgggggaggcttggtacagccgggggggtccctgagactctcctgtgcagcctctggattcaccttcagtagctacgacatacactgggtccgtcaagctacaggaaaaggtctggagtgggtctcagctattggtcctgctggtgacacatactatccaggctccgtgaagggccgattcaccatctccagagaaaatgccaagaactccttgtatcttcaaatgaacagcctgagagccggggacacggctgtgtattactgtgcaagaggtttgattacgtttggggggcttatcgccccgtttgactactggggccagggaaccctggtcaccgtctcctcagcctccaccaagggcccatcggtcttccccctggcaccctcctccaagagcacctctgggggcacagcggccctgggctgcctggtcaaggactacttccccgaaccggtgacggtgtcgtggaactcaggcgccctgaccagcggcgtgcacaccttcccggctgtcctacagtcctcaggactctactccctcagcagcgtggtgaccgtgccctccagcagcttgggcacccagacctacatctgcaacgtgaatcacaagcccagcaacaccaaggtggacaagaaagttgagcccaaatcttgtgacaaaactcacacatgcccaccgtgcccagcacctgaactcctggggggaccgtcagtcttcctcttccccccaaaacccaaggacaccctcatgatctcccggacccctgaggtcacatgcgtggtggtggacgtgagccacgaagaccctgaggtcaagttcaactggtacgtggacggcgtggaggtgcataatgccaagacaaagccgcgggaggagcagtacaacagcacgtaccgtgtggtcagcgtcctcaccgtcctgcaccaggactggctgaatggcaaggagtacaagtgcaaggtctccaacaaagccctcccagcccccatcgagaaaaccatctccaaagccaaagggcagccccgagaaccacaggtgtacaccctgcccccatcccgggatgagctgaccaagaaccaggtcagcctgacctgcctggtcaaaggcttctatcccagcgacatcgccgtggagtgggagagcaatgggcagccggagaacaactacaagaccacgcctcccgtgctggactccgacggctccttcttcctctacagcaagctcaccgtggacaagagcaggtggcagcaggggaacgtcttctcatgctccgtgatgcatgaggctctgcacaaccactacacgcagaagtccctctccctgtctccgggtaaatgagcggccgctaatcagccataccacatttgtagaggttttacttgctttaaaaaacctcccacacctccccctgaacctgaaacataaaatgaatgcaattgttgttgttaacttgtttattgcagcttataatggttacaaataaagcaatagcatcacaaatttcacaaataaagcatttttttcactgcattctagttgtggtttgtccaaactcatcaatgtatcttatcatgtctaccggtcctgcagggcccctctcttcatgtgagcaaaaggccagcaaaaggccaggaaccgtaaaaaggccgcgttgctggcgtttttccataggctccgcccccctgacgagcatcacaaaaatcgacgctcaagtcagaggtggcgaaacccgacaggactataaagataccaggcgtttccccctggaagctccctcgtgcgctctcctgttccgaccctgccgcttaccggatacctgtccgcctttctcccttcgggaagcgtggcgctttctcaatgctcacgctgtaggtatctcagttcggtgtaggtcgttcgctccaagctgggctgtgtgcacgaaccccccgttcagcccgaccgctgcgccttatccggtaactatcgtcttgagtccaacccggtaagacacgacttatcgccactggcagcagccactggtaacaggattagcagagcgaggtatgtaggcggtgctacagagttcttgaagtggtggcctaactacggctacactagaaggacagtatttggtatctgcgctctgctgaagccagttaccttcggaaaaagagttggtagctcttgatccggcaaacaaaccaccgctggtagcggtggtttttttgtttgcaagcagcagattacgcgcagaaaaaaaggatctcaagaagatcctttgatcttttctacggggtctgacgctcagtggaacgaaaactcacgttaagggattttggtcatgggcgcgcctcatactcctgcaggcatgagattatcaaaaaggatcttcacctagatccttttaaattaaaaatgaagttttaaatcaatctaaagtatatatgagtaaacttggtctgacagttaccaatgcttaatcagtgaggcacctatctcagcgatctgtctatttcgttcatccatagttgcctgactccccgtcgtgtagataactacgatacgggagggcttaccatctggccccagtgctgcaatgataccgcgagacccacgctcaccggctccagatttatcagcaataaaccagccagccggaagggccgagcgcagaagtggtcctgcaactttatccgcctccatccagtctattaattgttgccgggaagctagagtaagtagttcgccagttaatagtttgcgcaacgttgttgccattgctacaggcatcgtggtgtcacgctcgtcgtttggtatggcttcattcagctccggttcccaacgatcaaggcgagttacatgatcccccatgttgtgcaaaaaagcggttagctccttcggtcctccgatcgttgtcagaagtaagttggccgcagtgttatcactcatggttatggcagcactgcataattctcttactgtcatgccatccgtaagatgcttttctgtgactggtgagtactcaaccaagtcattctgagaatagtgtatgcggcgaccgagttgctcttgcccggcgtcaatacgggataataccgcgccacatagcagaactttaaaagtgctcatcattggaaaacgttcttcggggcgaaaactctcaaggatcttaccgctgttgagatccagttcgatgtaacccactcgtgcacccaactgatcttcagcatcttttactttcaccagcgtttctgggtgagcaaaaacaggaaggcaaaatgccgcaaaaaagggaataagggcgacacggaaatgttgaatactcatactcttcctttttcaatattattgaagcatttatcagggttattgtctcatgagcggatacatatttgaatgtatttagaaaaataaacaaataggggttccgcgcacatttccccgaaaagtgccacctgacgtcaggtaccaagcctaggcctccaaaaaagcctcctcactacttctggaatagctcagaggcagaggcggcctcggcctctgcataaataaaaaaaattagtcagccatggggcggagaatgggcggaactgggcggagttaggggcgggatgggcggagttaggggcgggactatggttgctgactaattgagatgcatgctttgcatacttctgcctgctggggagcctggggactttccacacctggttgctgactaattgagatgcatgctttgcatacttctgcctgctggggagcctggggactttccacaccggatccaccatggatagatccggaaagcctgaactcaccgcgacgtctgtcgagaagtttctgatcgaaaagttcgacagcgtctccgacctgatgcagctctcggagggcgaagaatctcgtgctttcagcttcgatgtaggagggcgtggatatgtcctgcgggtaaatagctgcgccgatggtttctacaaagatcgttatgtttatcggcactttgcatcggccgcgctcccgattccggaagtgcttgacattggggagttcagcgagagcctgacctattgcatctcccgccgtgcacagggtgtcacgttgcaagacctgcctgaaaccgaactgcccgctgttctgcagccggtcgcggaggccatggatgcgatcgctgcggccgatcttagccagacgagcgggttcggcccattcggaccgcaaggaatcggtcaatacactacatggcgtgatttcatatgcgcgattgctgatccccatgtgtatcactggcaaactgtgatggacgacaccgtcagtgcgtccgtcgcgcaggctctcgatgagctgatgctttgggccgaggactgccccgaagtccggcacctcgtgcacgcggatttcggctccaacaatgtcctgacggacaatggccgcataacagcggtcattgactggagcgaggcgatgttcggggattcccaatacgaggtcgccaacatcttcttctggaggccgtggttggcttgtatggagcagcagacgcgctacttcgagcggaggcatccggagcttgcaggatcgccgcggctccgggcgtatatgctccgcattggtcttgaccaactctatcagagcttggttgacggcaatttcgatgatgcagcttgggcgcagggtcgatgcgacgcaatcgtccgatccggagccgggactgtcgggcgtacacaaatcgcccgcagaagcgcggccgtctggaccgatggctgtgtagaagtactcgccgatagtggaaaccgacgccccagcactcgtccgagggcaaaggaatagacgcgtgctgtaagtctgcagaaattgatgatctattaaacaataaagatgtccactaaaatggaagtttttcctgtcatactttgttaagaagggtgagaacagagtacctacattttgaatggaaggattggagctacgggggtgggggtggggtgggattagataaatgcctgctctttactgaaggctctttactattgctttatgataatgtttcatagttggatatcataatttaaacaagcaaaaccaaattaagggccagctcattcctcccactcatgatctatggatctatagatctctcgtgcagctggggctctagggggtatccccacgcgccctgtagcggcgcattaagcgcggcgggtgtggtggttacgcgcagcgtgaccgctacacttgccagcgccctagcgcccgctcctttcgctttcttcccttcctttctcgccacgttcgccggctttccccgtcaagctctaaatcgggggctccctttagggttccgatttagtgctttacggcacctcgaccccaaaaaacttgattagggtgatggttcacgtagtgggccatcgccctgatagacggtttttcgccctttgacgttggagtccacgttctttaatagtggactcttgttccaaactggaacaacactcaaccctatctcggtctattcttttgatttataagggattttgccgatttcggcctattggttaaaaaatgagctgatttaacaaaaatttaacgcgaattaattctgtggaatgtgtgtcagttag

SEQ ID NO: 33 - DNA, 2272 bp, synthetic construct
  misc_feature 1..2272: note = Synthetic construct
  source 1..2272: mol_type = other DNA
tagttattaatagtaatcaattacggggtcattagttcatagcccatatatggagttccgcgttacataacttacggtaaatggcccgcctggctgaccgcccaacgacccccgcccattgacgtcaataatgacgtatgttcccatagtaacgccaatagggactttccattgacgtcaatgggtggagtatttacggtaaactgcccacttggcagtacatcaagtgtatcatatgccaagtacgccccctattgacgtcaatgacggtaaatggcccgcctggcattatgcccagtacatgaccttatgggactttcctacttggcagtacatctacgtattagtcatcgctattaccatggtgatgcggttttggcagtacatcaatgggcgtggatagcggtttgactcacggggatttccaagtctccaccccattgacgtcaatgggagtttgttttggcaccaaaatcaacgggactttccaaaatgtcgtaacaactccgccccattgacgcaaatgggcggtaggcgtgtacggtgggaggtctatataagcagagctcatgatagaagcactctactattcgtcgaccgatcctgagaacttcagggtgagtttggggacccttgattgttctttctttttcgctattgtaaaattcatgttatatggagggggcaaagttttcagggtgttgtttagaatgggaagatgtcccttgtatcaccatggaccctcatgataattttgtttctttcactttctactctgttgacaaccattgtctcctcttattttcttttcattttctgtaactttttcgttaaactttagcttgcatttgtaacgaatttttaaattcacttttgtttatttgtcagattgtaagtactttctctaatcacttttttttcaaggcaatcagggtatattatattgtacttcagcacagttttagagaacaattgttataattaaatgataaggtagaatatttctgcatataaattctggctggcgtggaaatattcttattggtagaaacaactacaccctggtcatcatcctgcctttctctttatggttacaatgatatacactgtttgagatgaggataaaatactctgagtccaaaccgggcccctctgctaaccatgttcatgccttcttctctttcctacagctcctgggcaacgtgctggttgttgtgctgtctcatcattttggcaaagaattaagcttatactcgagctctagattgggaacccgggtctctcgaattcgagatctccaccatgcacagacctagacgtcgtggaactcgtccacctccactggcactgctcgctgctctcctcctggctgcacgtggtgctgatgcagaaattgtgttgacgcagtctccaggcaccctgtctttgtctccaggggaaagagccaccctctcctgcagggccagtcagagtgttagcagcacctacttagcctggtaccagcagaaacctggccaggctcccaggctcctcatctatggtgcatccagcagggccactggcatcccagacaggttcagtggcagtgggtctgggacagacttcactctcaccatcagcagactggagcctgaagattttgcagtgtattactgtcagcattatgataactcacaaacgttcggccaagggaccaaggtggagatcaaacgaactgtggctgcaccatctgtcttcatcttcccgccatctgatgagcagttgaaatctggaactgcctctgttgtgtgcctgctgaataacttctatcccagagaggccaaagtacagtggaaggtggataacgccctccaatcgggtaactcccaggagagtgtcacagagcaggacagcaaggacagcacctacagcctcagcagcaccctgacgctgagcaaagcagactacgagaaacacaaagtctacgcctgcgaagtcacccatcagggcctgagctcgcccgtcacaaagagcttcaacaggggagagtgttaggcggccgctaatcagccataccacatttgtagaggttttacttgctttaaaaaacctcccacacctccccctgaacctgaaacataaaatgaatgcaattgttgttgttaacttgtttattgcagcttataatggttacaaataaagcaatagcatcacaaatttcacaaataaagcatttttttcactgcattctagttgtggtttgtccaaactcatcaatgtatcttatcatgtc

SEQ ID NO: 34 - DNA, 6335 bp, synthetic construct
  misc_feature 1..6335: note = Synthetic plasmid
  source 1..6335: mol_type = other DNA
tcgagctctagattgggaacccgggtctctcgaattcgagatctccaccatgcacagacctagacgtcgtggaactcgtccacctccactggcactgctcgctgctctcctcctggctgcacgtggtgctgatgcagaaattgtgttgacgcagtctccaggcaccctgtctttgtctccaggggaaagagccaccctctcctgcagggccagtcagagtgttagcagcacctacttagcctggtaccagcagaaacctggccaggctcccaggctcctcatctatggtgcatccagcagggccactggcatcccagacaggttcagtggcagtgggtctgggacagacttcactctcaccatcagcagactggagcctgaagattttgcagtgtattactgtcagcattatgataactcacaaacgttcggccaagggaccaaggtggagatcaaacgaactgtggctgcaccatctgtcttcatcttcccgccatctgatgagcagttgaaatctggaactgcctctgttgtgtgcctgctgaataacttctatcccagagaggccaaagtacagtggaaggtggataacgccctccaatcgggtaactcccaggagagtgtcacagagcaggacagcaaggacagcacctacagcctcagcagcaccctgacgctgagcaaagcagactacgagaaacacaaagtctacgcctgcgaagtcacccatcagggcctgagctcgcccgtcacaaagagcttcaacaggggagagtgttaggcggccgctaatcagccataccacatttgtagaggttttacttgctttaaaaaacctcccacacctccccctgaacctgaaacataaaatgaatgcaattgttgttgttaacttgtttattgcagcttataatggttacaaataaagcaatagcatcacaaatttcacaaataaagcatttttttcactgcattctagttgtggtttgtccaaactcatcaatgtatcttatcatgtctaccggtagggcccctctcttcatgtgagcaaaaggccagcaaaaggccaggaaccgtaaaaaggccgcgttgctggcgtttttccataggctccgcccccctgacgagcatcacaaaaatcgacgctcaagtcagaggtggcgaaacccgacaggactataaagataccaggcgtttccccctggaagctccctcgtgcgctctcctgttccgaccctgccgcttaccggatacctgtccgcctttctcccttcgggaagcgtggcgctttctcaatgctcacgctgtaggtatctcagttcggtgtaggtcgttcgctccaagctgggctgtgtgcacgaaccccccgttcagcccgaccgctgcgccttatccggtaactatcgtcttgagtccaacccggtaagacacgacttatcgccactggcagcagccactggtaacaggattagcagagcgaggtatgtaggcggtgctacagagttcttgaagtggtggcctaactacggctacactagaaggacagtatttggtatctgcgctctgctgaagccagttaccttcggaaaaagagttggtagctcttgatccggcaaacaaaccaccgctggtagcggtggtttttttgtttgcaagcagcagattacgcgcagaaaaaaaggatctcaagaagatcctttgatcttttctacggggtctgacgctcagtggaacgaaaactcacgttaagggattttggtcatgggcgcgggcatgagattatcaaaaaggatcttcacctagatccttttaaattaaaaatgaagttttaaatcaatctaaagtatatatgagtaaacttggtctgacagttaccaatgcttaatcagtgaggcacctatctcagcgatctgtctatttcgttcatccatagttgcctgactccccgtcgtgtagataactacgatacgggagggcttaccatctggccccagtgctgcaatgataccgcgagacccacgctcaccggctccagatttatcagcaataaaccagccagccggaagggccgagcgcagaagtggtcctgcaactttatccgcctccatccagtctattaattgttgccgggaagctagagtaagtagttcgccagttaatagtttgcgcaacgttgttgccattgctacaggcatcgtggtgtcacgctcgtcgtttggtatggcttcattcagctccggttcccaacgatcaaggcgagttacatgatcccccatgttgtgcaaaaaagcggttagctccttcggtcctccgatcgttgtcagaagtaagttggccgcagtgttatcactcatggttatggcagcactgcataattctcttactgtcatgccatccgtaagatgcttttctgtgactggtgagtactcaaccaagtcattctgagaatagtgtatgcggcgaccgagttgctcttgcccggcgtcaatacgggataataccgcgccacatagcagaactttaaaagtgctcatcattggaaaacgttcttcggggcgaaaactctcaaggatcttaccgctgttgagatccagttcgatgtaacccactcgtgcacccaactgatcttcagcatcttttactttcaccagcgtttctgggtgagcaaaaacaggaaggcaaaatgccgcaaaaaagggaataagggcgacacggaaatgttgaatactcatactcttcctttttcaatattattgaagcatttatcagggttattgtctcatgagcggatacatatttgaatgtatttagaaaaataaacaaataggggttccgcgcacatttccccgaaaagtgccacctgacgtcaggtacacttaggcgcgccattagagttcctgcaggctacatggtaccaagcctaggcctccaaaaaagcctcctcactacttctggaatagctcagaggcagaggcggcctcggcctctgcataaataaaaaaaattagtcagccatggggcggagaatgggcggaactgggcggagttaggggcgggatgggcggagttaggggcgggactatggttgctgactaattgagatgcatgctttgcatacttctgcctgctggggagcctggggactttccacacctggttgctgactaattgagatgcatgctttgcatacttctgcctgctggggagcctggggactttccacaccggatccaccatggatagatccggaaagcctgaactcaccgcgacgtctgtcgagaagtttctgatcgaaaagttcgacagcgtctccgacctgatgcagctctcggagggcgaagaatctcgtgctttcagcttcgatgtaggagggcgtggatatgtcctgcgggtaaatagctgcgccgatggtttctacaaagatcgttatgtttatcggcactttgcatcggccgcgctcccgattccggaagtgcttgacattggggagttcagcgagagcctgacctattgcatctcccgccgtgcacagggtgtcacgttgcaagacctgcctgaaaccgaactgcccgctgttctgcagccggtcgcggaggccatggatgcgatcgctgcggccgatcttagccagacgagcgggttcggcccattcggaccgcaaggaatcggtcaatacactacatggcgtgatttcatatgcgcgattgctgatccccatgtgtatcactggcaaactgtgatggacgacaccgtcagtgcgtccgtcgcgcaggctctcgatgagctgatgctttgggccgaggactgccccgaagtccggcacctcgtgcacgcggatttcggctccaacaatgtcctgacggacaatggccgcataacagcggtcattgactggagcgaggcgatgttcggggattcccaatacgaggtcgccaacatcttcttctggaggccgtggttggcttgtatggagcagcagacgcgctacttcgagcggaggcatccggagcttgcaggatcgccgcggctccgggcgtatatgctccgcattggtcttgaccaactctatcagagcttggttgacggcaatttcgatgatgcagcttgggcgcagggtcgatgcgacgcaatcgtccgatccggagccgggactgtcgggcgtacacaaatcgcccgcagaagcgcggccgtctggaccgatggctgtgtagaagtactcgccgatagtggaaaccgacgccccagcactcgtccgagggcaaaggaatagacgcgtgctgtaagtctgcagaaattgatgatctattaaacaataaagatgtccactaaaatggaagtttttcctgtcatactttgttaagaagggtgagaacagagtacctacattttgaatggaaggattggagctacgggggtgggggtggggtgggattagataaatgcctgctctttactgaaggctctttactattgctttatgataatgtttcatagttggatatcataatttaaacaagcaaaaccaaattaagggccagctcattcctcccactcatgatctatggatctatagatctctcgtgcagctggggctctagggggtatccccacgcgccctgtagcggcgcattaagcgcggcgggtgtggtggttacgcgcagcgtgaccgctacacttgccagcgccctagcgcccgctcctttcgctttcttcccttcctttctcgccacgttcgccggctttccccgtcaagctctaaatcgggggctccctttagggttccgatttagtgctttacggcacctcgaccccaaaaaacttgattagggtgatggttcacgtagtgggccatcgccctgatagacggtttttcgccctttgacgttggagtccacgttctttaatagtggactcttgttccaaactggaacaacactcaaccctatctcggtctattcttttgatttataagggattttgccgatttcggcctattggttaaaaaatgagctgatttaacaaaaatttaacgcgaattaattctgtggaatgtgtgtcagttagtcgcgatgtgtgactagttagttattaatagtaatcaattacggggtcattagttcatagcccatatatggagttccgcgttacataacttacggtaaatggcccgcctggctgaccgcccaacgacccccgcccattgacgtcaataatgacgtatgttcccatagtaacgccaatagggactttccattgacgtcaatgggtggagtatttacggtaaactgcccacttggcagtacatcaagtgtatcatatgccaagtacgccccctattgacgtcaatgacggtaaatggcccgcctggcattatgcccagtacatgaccttatgggactttcctacttggcagtacatctacgtattagtcatcgctattaccatggtgatgcggttttggcagtacatcaatgggcgtggatagcggtttgactcacggggatttccaagtctccaccccattgacgtcaatgggagtttgttttggcaccaaaatcaacgggactttccaaaatgtcgtaacaactccgccccattgacgcaaatgggcggtaggcgtgtacggtgggaggtctatataagcagagctcatgatagaagcactctactattcgtcgaccgatcctgagaacttcagggtgagtttggggacccttgattgttctttctttttcgctattgtaaaattcatgttatatggagggggcaaagttttcagggtgttgtttagaatgggaagatgtcccttgtatcaccatggaccctcatgataattttgtttctttcactttctactctgttgacaaccattgtctcctcttattttcttttcattttctgtaactttttcgttaaactttagcttgcatttgtaacgaatttttaaattcacttttgtttatttgtcagattgtaagtactttctctaatcacttttttttcaaggcaatcagggtatattatattgtacttcagcacagttttagagaacaattgttataattaaatgataaggtagaatatttctgcatataaattctggctggcgtggaaatattcttattggtagaaacaactacaccctggtcatcatcctgcctttctctttatggttacaatgatatacactgtttgagatgaggataaaatactctgagtccaaaccgggcccctctgctaaccatgttcatgccttcttctctttcctacagctcctgggcaacgtgctggttgttgtgctgtctcatcattttggcaaagaattaagcttatac

SEQ ID NO: 35 - protein, 449 aa, Homo sapiens
QVQLQQSGAGLLKPSETLSLTCTVYGGSFSIHHWTWIRHPPGKGLEWIGEINHRGSTNYNPSLKSRVTISIDTSKNQFSLKLSAVTAADTAVYYCARGLRFLDWLSSYFDYWGQGTLVTVSSASTKGPSVFPLAPCSRSTSESTAALGCLVKDYFPEPVTVSWNSGALTSGVHTFPAVLQSSGLYSLSSVVTVPSSSLGTKTYTCNVDHKPSNTKVDKRVESKYGPPCPPCPAPEFLGGPSVFLFPPKPKDTLMISRTPEVTCVVVDVSQEDPEVQFNWYVDGVEVHNAKTKPREEQFNSTYRVVSVLTVLHQDWLNGKEYKCKVSNKGLPSSIEKTISKAKGQPREPQVYTLPPSQEEMTKNQVSLTCLVKGFYPSDIAVEWESNGQPENNYKTTPPVLDSDGSFFLYSRLTVDKSRWQEGNVFSCSVMHEALHNHYTQKSLSLSLGK

SEQ ID NO: 36 - protein, 103 aa, Homo sapiens
QSGAGLLKPSETLSLTCTVYGGSFSIHHWTWIRHPPGKGLEWIGEINHRGSTNYNPSLKSRVTISIDTSKNQFSLKLSAVTAADTAVYYCARGLRFLDWLSSY

SEQ ID NO: 37 - protein, 214 aa, Homo sapiens
DIQMTQSPSSLSASVGDRVTITCRASQGISDYLAWYQQKPGKVPNLLIYAASALQSGVPSRFSGSGSGTDFTLTISSLQPEDVATYYCQNYNTAPLTFGGGTKVEIKRTVAAPSVFIFPPSDEQLKSGTASVVCLLNNFYPREAKVQWKVDNALQSGNSQESVTEQDSKDSTYSLSSTLTLSKADYEKHKVYACEVTHQGLSSPVTKSFNRGEC

SEQ ID NO: 38 - protein, 107 aa, Homo sapiens
IQMTQSPSSLSASVGDRVTITCRASQGISDYLAWYQQKPGKVPNLLIYAASALQSGVPSRFSGSGSGTDFTLTISSLQPEDVATYYCQNYNTAPLTFGGGTKVEIKR

SEQ ID NO: 39 - DNA, 2977 bp, synthetic construct
  misc_feature 1..2977: note = Synthetic construct
  source 1..2977: mol_type = other DNA
tagttattaatagtaatcaattacggggtcattagttcatagcccatatatggagttccgcgttacataacttacggtaaatggcccgcctggctgaccgcccaacgacccccgcccattgacgtcaataatgacgtatgttcccatagtaacgccaatagggactttccattgacgtcaatgggtggagtatttacggtaaactgcccacttggcagtacatcaagtgtatcatatgccaagtacgccccctattgacgtcaatgacggtaaatggcccgcctggcattatgcccagtacatgaccttatgggactttcctacttggcagtacatctacgtattagtcatcgctattaccatggtgatgcggttttggcagtacatcaatgggcgtggatagcggtttgactcacggggatttccaagtctccaccccattgacgtcaatgggagtttgttttggcaccaaaatcaacgggactttccaaaatgtcgtaacaactccgccccattgacgcaaatgggcggtaggcgtgtacggtgggaggtctatataagcagagctcatgatagaagcactctactattcgtcgaccgatcctgagaacttcagggtgagtttggggacccttgattgttctttctttttcgctattgtaaaattcatgttatatggagggggcaaagttttcagggtgttgtttagaatgggaagatgtcccttgtatcaccatggaccctcatgataattttgtttctttcactttctactctgttgacaaccattgtctcctcttattttcttttcattttctgtaactttttcgttaaactttagcttgcatttgtaacgaatttttaaattcacttttgtttatttgtcagattgtaagtactttctctaatcacttttttttcaaggcaatcagggtatattatattgtacttcagcacagttttagagaacaattgttataattaaatgataaggtagaatatttctgcatataaattctggctggcgtggaaatattcttattggtagaaacaactacaccctggtcatcatcctgcctttctctttatggttacaatgatatacactgtttgagatgaggataaaatactctgagtccaaaccgggcccctctgctaaccatgttcatgccttcttctctttcctacagctcctgggcaacgtgctggttgttgtgctgtctcatcattttggcaaagaattaagcttatactcgagctctagattgggaacccgggtctctcgaattcgagatctccaccatgcacagacctagacgtcgtggaactcgtccacctccactggcactgctcgctgctctcctcctggctgcacgtggtgctgatgcacaggtacagctgcagcagtcgggcgcaggactgttgaagccttcggagaccctgtccctcacctgcactgtctatggtggatccttcagtattcatcactggacctggatccgccatcccccagggaaggggctggagtggattggggagatcaatcatcgtggaagcaccaactacaacccgtccctcaagagtcgagtcaccatatcaatagacacgtccaagaaccagttctccctgaagctgagcgctgtgaccgccgcggacacggctgtatattactgtgcgagaggcttacgatttttggactggttatcgtcctactttgactactggggccagggaaccctggtcaccgtctcctcagcctccaccaagggcccatcggtcttccccctggcgccctgctccaggagcacctccgagagcacagccgccctgggctgcctggtcaaggactacttccccgaaccggtgacggtgtcgtggaactcaggcgccctgaccagcggcgtgcacaccttcccggctgtcctacagtcctcaggactctactccctcagcagcgtggtgaccgtgccctccagcagcttgggcacgaagacctacacctgcaacgtagatcacaagcccagcaacaccaaggtggacaagagagttgagtccaaatatggtcccccatgcccaccctgcccagcacctgagttcctggggggaccatcagtcttcctgttccccccaaaacccaaggacactctcatgatctcccggacccctgaggtcacgtgcgtggtggtggacgtgagccaggaagaccccgaggtccagttcaactggtacgtggatggcgtggaggtgcataatgccaagacaaagccgcgggaggagcagttcaacagcacgtaccgtgtggtcagcgtcctcaccgtcctgcaccaggactggctgaacggcaaggagtacaagtgcaaggtctccaacaaaggcctcccgtcctccatcgagaaaaccatctccaaagccaaagggcagccccgagagccacaggtgtacaccctgcccccatcccaggaggagatgaccaagaaccaggtcagcctgacctgcctggtcaaaggcttctaccccagcgacatcgccgtggagtgggagagcaatgggcagccggagaacaactacaagaccacgcctcccgtgctggactccgacggctccttcttcctctacagcaggctcaccgtggacaagagcaggtggcaggaggggaatgtcttctcatgctccgtgatgcatgaggctctgcacaaccactacacacagaagtccctctccctgtctctgggtaaatgagcggccgctaatcagccataccacatttgtagaggttttacttgctttaaaaaacctcccacacctccccctgaacctgaaacataaaatgaatgcaattgttgttgttaacttgtttattgcagcttataatggttacaaataaagcaatagcatcacaaatttcacaaataaagcatttttttcactgcattctagttgtggtttgtccaaactcatcaatgtatcttatcatgtc

SEQ ID NO: 40 - DNA, 7019 bp, synthetic construct
  misc_feature 1..7019: note = Synthetic plasmid
  source 1..7019: mol_type = other DNA
tcgcgatgtgtgactagttagttattaatagtaatcaattacggggtcattagttcatagcccatatatggagttccgcgttacataacttacggtaaatggcccgcctggctgaccgcccaacgacccccgcccattgacgtcaataatgacgtatgttcccatagtaacgccaatagggactttccattgacgtcaatgggtggagtatttacggtaaactgcccacttggcagtacatcaagtgtatcatatgccaagtacgccccctattgacgtcaatgacggtaaatggcccgcctggcattatgcccagtacatgaccttatgggactttcctacttggcagtacatctacgtattagtcatcgctattaccatggtgatgcggttttggcagtacatcaatgggcgtggatagcggtttgactcacggggatttccaagtctccaccccattgacgtcaatgggagtttgttttggcaccaaaatcaacgggactttccaaaatgtcgtaacaactccgccccattgacgcaaatgggcggtaggcgtgtacggtgggaggtctatataagcagagctcatgatagaagcactctactattcgtcgaccgatcctgagaacttcagggtgagtttggggacccttgattgttctttctttttcgctattgtaaaattcatgttatatggagggggcaaagttttcagggtgttgtttagaatgggaagatgtcccttgtatcaccatggaccctcatgataattttgtttctttcactttctactctgttgacaaccattgtctcctcttattttcttttcattttctgtaactttttcgttaaactttagcttgcatttgtaacgaatttttaaattcacttttgtttatttgtcagattgtaagtactttctctaatcacttttttttcaaggcaatcagggtatattatattgtacttcagcacagttttagagaacaattgttataattaaatgataaggtagaatatttctgcatataaattctggctggcgtggaaatattcttattggtagaaacaactacaccctggtcatcatcctgcctttctctttatggttacaatgatatacactgtttgagatgaggataaaatactctgagtccaaaccgggcccctctgctaaccatgttcatgccttcttctctttcctacagctcctgggcaacgtgctggttgttgtgctgtctcatcattttggcaaagaattaagcttatactcgagctctagattgggaacccgggtctctcgaattcgagatctccaccatgcacagacctagacgtcgtggaactcgtccacctccactggcactgctcgctgctctcctcctggctgcacgtggtgctgatgcacaggtacagctgcagcagtcgggcgcaggactgttgaagccttcggagaccctgtccctcacctgcactgtctatggtggatccttcagtattcatcactggacctggatccgccatcccccagggaaggggctggagtggattggggagatcaatcatcgtggaagcaccaactacaacccgtccctcaagagtcgagtcaccatatcaatagacacgtccaagaaccagttctccctgaagctgagcgctgtgaccgccgcggacacggctgtatattactgtgcgagaggcttacgatttttggactggttatcgtcctactttgactactggggccagggaaccctggtcaccgtctcctcagcctccaccaagggcccatcggtcttccccctggcgccctgctccaggagcacctccgagagcacagccgccctgggctgcctggtcaaggactacttccccgaaccggtgacggtgtcgtggaactcaggcgccctgaccagcggcgtgcacaccttcccggctgtcctacagtcctcaggactctactccctcagcagcgtggtgaccgtgccctccagcagcttgggcacgaagacctacacctgcaacgtagatcacaagcccagcaacaccaaggtggacaagagagttgagtccaaatatggtcccccatgcccaccctgcccagcacctgagttcctggggggaccatcagtcttcctgttccccccaaaacccaaggacactctcatgatctcccggacccctgaggtcacgtgcgtggtggtggacgtgagccaggaagaccccgaggtccagttcaactggtacgtggatggcgtggaggtgcataatgccaagacaaagccgcgggaggagcagttcaacagcacgtaccgtgtggtcagcgtcctcaccgtcctgcaccaggactggctgaacggcaaggagtacaagtgcaaggtctccaacaaaggcctcccgtcctccatcgagaaaaccatctccaaagccaaagggcagccccgagagccacaggtgtacaccctgcccccatcccaggaggagatgaccaagaaccaggtcagcctgacctgcctggtcaaaggcttctaccccagcgacatcgccgtggagtgggagagcaatgggcagccggagaacaactacaagaccacgcctcccgtgctggactccgacggctccttcttcctctacagcaggctcaccgtggacaagagcaggtggcaggaggggaatgtcttctcatgctccgtgatgcatgaggctctgcacaaccactacacacagaagtccctctccctgtctctgggtaaatgagcggccgctaatcagccataccacatttgtagaggttttacttgctttaaaaaacctcccacacctccccctgaacctgaaacataaaatgaatgcaattgttgttgttaacttgtttattgcagcttataatggttacaaataaagcaatagcatcacaaatttcacaaataaagcatttttttcactgcattctagttgtggtttgtccaaactcatcaatgtatcttatcatgtctaccggtcctgcagggcccctctcttcatgtgagcaaaaggccagcaaaaggccaggaaccgtaaaaaggccgcgttgctggcgtttttccataggctccgcccccctgacgagcatcacaaaaatcgacgctcaagtcagaggtggcgaaacccgacaggactataaagataccaggcgtttccccctggaagctccctcgtgcgctctcctgttccgaccctgccgcttaccggatacctgtccgcctttctcccttcgggaagcgtggcgctttctcaatgctcacgctgtaggtatctcagttcggtgtaggtcgttcgctccaagctgggctgtgtgcacgaaccccccgttcagcccgaccgctgcgccttatccggtaactatcgtcttgagtccaacccggtaagacacgacttatcgccactggcagcagccactggtaacaggattagcagagcgaggtatgtaggcggtgctacagagttcttgaagtggtggcctaactacggctacactagaaggacagtatttggtatctgcgctctgctgaagccagttaccttcggaaaaagagttggtagctcttgatccggcaaacaaaccaccgctggtagcggtggtttttttgtttgcaagcagcagattacgcgcagaaaaaaaggatctcaagaagatcctttgatcttttctacggggtctgacgctcagtggaacgaaaactcacgttaagggattttggtcatgggcgcgcctcatactcctgcaggcatgagattatcaaaaaggatcttcacctagatccttttaaattaaaaatgaagttttaaatcaatctaaagtatatatgagtaaacttggtctgacagttaccaatgcttaatcagtgaggcacctatctcagcgatctgtctatttcgttcatccatagttgcctgactccccgtcgtgtagataactacgatacgggagggcttaccatctggccccagtgctgcaatgataccgcgagacccacgctcaccggctccagatttatcagcaataaaccagccagccggaagggccgagcgcagaagtggtcctgcaactttatccgcctccatccagtctattaattgttgccgggaagctagagtaagtagttcgccagttaatagtttgcgcaacgttgttgccattgctacaggcatcgtggtgtcacgctcgtcgtttggtatggcttcattcagctccggttcccaacgatcaaggcgagttacatgatcccccatgttgtgcaaaaaagcggttagctccttcggtcctccgatcgttgtcagaagtaagttggccgcagtgttatcactcatggttatggcagcactgcataattctcttactgtcatgccatccgtaagatgcttttctgtgactggtgagtactcaaccaagtcattctgagaatagtgtatgcggcgaccgagttgctcttgcccggcgtcaatacgggataataccgcgccacatagcagaactttaaaagtgctcatcattggaaaacgttcttcggggcgaaaactctcaaggatcttaccgctgttgagatccagttcgatgtaacccactcgtgcacccaactgatcttcagcatcttttactttcaccagcgtttctgggtgagcaaaaacaggaaggcaaaatgccgcaaaaaagggaataagggcgacacggaaatgttgaatactcatactcttcctttttcaatattattgaagcatttatcagggttattgtctcatgagcggatacatatttgaatgtatttagaaaaataaacaaataggggttccgcgcacatttccccgaaaagtgccacctgacgtcaggtaccaagcctaggcctccaaaaaagcctcctcactacttctggaatagctcagaggcagaggcggcctcggcctctgcataaataaaaaaaattagtcagccatggggcggagaatgggcggaactgggcggagttaggggcgggatgggcggagttaggggcgggactatggttgctgactaattgagatgcatgctttgcatacttctgcctgctggggagcctggggactttccacacctggttgctgactaattgagatgcatgctttgcatacttctgcctgctggggagcctggggactttccacaccggatccaccatggatagatccggaaagcctgaactcaccgcgacgtctgtcgagaagtttctgatcgaaaagttcgacagcgtctccgacctgatgcagctctcggagggcgaagaatctcgtgctttcagcttcgatgtaggagggcgtggatatgtcctgcgggtaaatagctgcgccgatggtttctacaaagatcgttatgtttatcggcactttgcatcggccgcgctcccgattccggaagtgcttgacattggggagttcagcgagagcctgacctattgcatctcccgccgtgcacagggtgtcacgttgcaagacctgcctgaaaccgaactgcccgctgttctgcagccggtcgcggaggccatggatgcgatcgctgcggccgatcttagccagacgagcgggttcggcccattcggaccgcaaggaatcggtcaatacactacatggcgtgatttcatatgcgcgattgctgatccccatgtgtatcactggcaaactgtgatggacgacaccgtcagtgcgtccgtcgcgcaggctctcgatgagctgatgctttgggccgaggactgccccgaagtccggcacctcgtgcacgcggatttcggctccaacaatgtcctgacggacaatggccgcataacagcggtcattgactggagcgaggcgatgttcggggattcccaatacgaggtcgccaacatcttcttctggaggccgtggttggcttgtatggagcagcagacgcgctacttcgagcggaggcatccggagcttgcaggatcgccgcggctccgggcgtatatgctccgcattggtcttgaccaactctatcagagcttggttgacggcaatttcgatgatgcagcttgggcgcagggtcgatgcgacgcaatcgtccgatccggagccgggactgtcgggcgtacacaaatcgcccgcagaagcgcggccgtctggaccgatggctgtgtagaagtactcgccgatagtggaaaccgacgccccagcactcgtccgagggcaaaggaatagacgcgtgctgtaagtctgcagaaattgatgatctattaaacaataaagatgtccactaaaatggaagtttttcctgtcatactttgttaagaagggtgagaacagagtacctacattttgaatggaaggattggagctacgggggtgggggtggggtgggattagataaatgcctgctctttactgaaggctctttactattgctttatgataatgtttcatagttggatatcataatttaaacaagcaaaaccaaattaagggccagctcattcctcccactcatgatctatggatctatagatctctcgtgcagctggggctctagggggtatccccacgcgccctgtagcggcgcattaagcgcggcgggtgtggtggttacgcgcagcgtgaccgctacacttgccagcgccctagcgcccgctcctttcgctttcttcccttcctttctcgccacgttcgccggctttccccgtcaagctctaaatcgggggctccctttagggttccgatttagtgctttacggcacctcgaccccaaaaaacttgattagggtgatggttcacgtagtgggccatcgccctgatagacggtttttcgccctttgacgttggagtccacgttctttaatagtggactcttgttccaaactggaacaacactcaaccctatctcggtctattcttttgatttataagggattttgccgatttcggcctattggttaaaaaatgagctgatttaacaaaaatttaacgcgaattaattctgtggaatgtgtgtcagttag

SEQ ID NO: 41 - DNA, 2272 bp, synthetic construct
  misc_feature 1..2272: note = Synthetic construct
  source 1..2272: mol_type = other DNA
tagttattaatagtaatcaattacggggtcattagttcatagcccatatatggagttccgcgttacataacttacggtaaatggcccgcctggctgaccgcccaacgacccccgcccattgacgtcaataatgacgtatgttcccatagtaacgccaatagggactttccattgacgtcaatgggtggagtatttacggtaaactgcccacttggcagtacatcaagtgtatcatatgccaagtacgccccctattgacgtcaatgacggtaaatggcccgcctggcattatgcccagtacatgaccttatgggactttcctacttggcagtacatctacgtattagtcatcgctattaccatggtgatgcggttttggcagtacatcaatgggcgtggatagcggtttgactcacggggatttccaagtctccaccccattgacgtcaatgggagtttgttttggcaccaaaatcaacgggactttccaaaatgtcgtaacaactccgccccattgacgcaaatgggcggtaggcgtgtacggtgggaggtctatataagcagagctcatgatagaagcactctactattcgtcgaccgatcctgagaacttcagggtgagtttggggacccttgattgttctttctttttcgctattgtaaaattcatgttatatggagggggcaaagttttcagggtgttgtttagaatgggaagatgtcccttgtatcaccatggaccctcatgataattttgtttctttcactttctactctgttgacaaccattgtctcctcttattttcttttcattttctgtaactttttcgttaaactttagcttgcatttgtaacgaatttttaaattcacttttgtttatttgtcagattgtaagtactttctctaatcacttttttttcaaggcaatcagggtatattatattgtacttcagcacagttttagagaacaattgttataattaaatgataaggtagaatatttctgcatataaattctggctggcgtggaaatattcttattggtagaaacaactacaccctggtcatcatcctgcctttctctttatggttacaatgatatacactgtttgagatgaggataaaatactctgagtccaaaccgggcccctctgctaaccatgttcatgccttcttctctttcctacagctcctgggcaacgtgctggttgttgtgctgtctcatcattttggcaaagaattaagcttatactcgagctctagattgggaacccgggtctctcgaattcgagatctccaccatgcacagacctagacgtcgtggaactcgtccacctccactggcactgctcgctgctctcctcctggctgcacgtggtgctgatgcagacatccagatgacccagtctccatcctccctgtctgcatctgtaggagacagagtcaccatcacttgccgggcgagtcagggcattagcgattatttagcctggtatcagcagaaaccagggaaagttcctaacctcctgatctatgctgcgtccgctttacaatcaggggtcccatctcgtttcagtggcagtggatctgggacagatttcactctcaccatcagcagcctgcagcctgaggatgttgcaacttattactgtcaaaattataacactgccccgctcactttcggcggggggaccaaggtggaaatcaaacgaactgtggctgcaccatctgtcttcatcttcccgccatctgatgagcagttgaaatctggaactgcctctgttgtgtgcctgctgaataacttctatcccagagaggccaaagtacagtggaaggtggataacgccctccaatcgggtaactcccaggagagtgtcacagagcaggacagcaaggacagcacctacagcctcagcagcaccctgacgctgagcaaagcagactacgagaaacacaaagtctacgcctgcgaagtcacccatcagggcctgagctcgcccgtcacaaagagcttcaacaggggagagtgttaggcggccgctaatcagccataccacatttgtagaggttttacttgctttaaaaaacctcccacacctccccctgaacctgaaacataaaatgaatgcaattgttgttgttaacttgtttattgcagcttataatggttacaaataaagcaatagcatcacaaatttcacaaataaagcatttttttcactgcattctagttgtggtttgtccaaactcatcaatgtatcttatcatgtc

SEQ ID NO: 42 - DNA, 6335 bp, synthetic construct
  misc_feature 1..6335: note = Synthetic plasmid
  source 1..6335: mol_type = other DNA
tcgagctctagattgggaacccgggtctctcgaattcgagatctccaccatgcacagacctagacgtcgtggaactcgtccacctccactggcactgctcgctgctctcctcctggctgcacgtggtgctgatgcagacatccagatgacccagtctccatcctccctgtctgcatctgtaggagacagagtcaccatcacttgccgggcgagtcagggcattagcgattatttagcctggtatcagcagaaaccagggaaagttcctaacctcctgatctatgctgcgtccgctttacaatcaggggtcccatctcgtttcagtggcagtggatctgggacagatttcactctcaccatcagcagcctgcagcctgaggatgttgcaacttattactgtcaaaattataacactgccccgctcactttcggcggggggaccaaggtggaaatcaaacgaactgtggctgcaccatctgtcttcatcttcccgccatctgatgagcagttgaaatctggaactgcctctgttgtgtgcctgctgaataacttctatcccagagaggccaaagtacagtggaaggtggataacgccctccaatcgggtaactcccaggagagtgtcacagagcaggacagcaaggacagcacctacagcctcagcagcaccctgacgctgagcaaagcagactacgagaaacacaaagtctacgcctgcgaagtcacccatcagggcctgagctcgcccgtcacaaagagcttcaacaggggagagtgttaggcggccgctaatcagccataccacatttgtagaggttttacttgctttaaaaaacctcccacacctccccctgaacctgaaacataaaatgaatgcaattgttgttgttaacttgtttattgcagcttataatggttacaaataaagcaatagcatcacaaatttcacaaataaagcatttttttcactgcattctagttgtggtttgtccaaactcatcaatgtatcttatcatgtctaccggtagggcccctctcttcatgtgagcaaaaggccagcaaaaggccaggaaccgtaaaaaggccgcgttgctggcgtttttccataggctccgcccccctgacgagcatcacaaaaatcgacgctcaagtcagaggtggcgaaacccgacaggactataaagataccaggcgtttccccctggaagctccctcgtgcgctctcctgttccgaccctgccgcttaccggatacctgtccgcctttctcccttcgggaagcgtggcgctttctcaatgctcacgctgtaggtatctcagttcggtgtaggtcgttcgctccaagctgggctgtgtgcacgaaccccccgttcagcccgaccgctgcgccttatccggtaactatcgtcttgagtccaacccggtaagacacgacttatcgccactggcagcagccactggtaacaggattagcagagcgaggtatgtaggcggtgctacagagttcttgaagtggtggcctaactacggctacactagaaggacagtatttggtatctgcgctctgctgaagccagttaccttcggaaaaagagttggtagctcttgatccggcaaacaaaccaccgctggtagcggtggtttttttgtttgcaagcagcagattacgcgcagaaaaaaaggatctcaagaagatcctttgatcttttctacggggtctgacgctcagtggaacgaaaactcacgttaagggattttggtcatgggcgcgggcatgagattatcaaaaaggatcttcacctagatccttttaaattaaaaatgaagttttaaatcaatctaaagtatatatgagtaaacttggtctgacagttaccaatgcttaatcagtgaggcacctatctcagcgatctgtctatttcgttcatccatagttgcctgactccccgtcgtgtagataactacgatacgggagggcttaccatctggccccagtgctgcaatgataccgcgagacccacgctcaccggctccagatttatcagcaataaaccagccagccggaagggccgagcgcagaagtggtcctgcaactttatccgcctccatccagtctattaattgttgccgggaagctagagtaagtagttcgccagttaatagtttgcgcaacgttgttgccattgctacaggcatcgtggtgtcacgctcgtcgtttggtatggcttcattcagctccggttcccaacgatcaaggcgagttacatgatcccccatgttgtgcaaaaaagcggttagctccttcggtcctccgatcgttgtcagaagtaagttggccgcagtgttatcactcatggttatggcagcactgcataattctcttactgtcatgccatccgtaagatgcttttctgtgactggtgagtactcaaccaagtcattctgagaatagtgtatgcggcgaccgagttgctcttgcccggcgtcaatacgggataataccgcgccacatagcagaactttaaaagtgctcatcattggaaaacgttcttcggggcgaaaactctcaaggatcttaccgctgttgagatccagttcgatgtaacccactcgtgcacccaactgatcttcagcatcttttactttcaccagcgtttctgggtgagcaaaaacaggaaggcaaaatgccgcaaaaaagggaataagggcgacacggaaatgttgaatactcatactcttcctttttcaatattattgaagcatttatcagggttattgtctcatgagcggatacatatttgaatgtatttagaaaaataaacaaataggggttccgcgcacatttccccgaaaagtgccacctgacgtcaggtacacttaggcgcgccattagagttcctgcaggctacatggtaccaagcctaggcctccaaaaaagcctcctcactacttctggaatagctcagaggcagaggcggcctcggcctctgcataaataaaaaaaattagtcagccatggggcggagaatgggcggaactgggcggagttaggggcgggatgggcggagttaggggcgggactatggttgctgactaattgagatgcatgctttgcatacttctgcctgctggggagcctggggactttccacacctggttgctgactaattgagatgcatgctttgcatacttctgcctgctggggagcctggggactttccacaccggatccaccatggatagatccggaaagcctgaactcaccgcgacgtctgtcgagaagtttctgatcgaaaagttcgacagcgtctccgacctgatgcagctctcggagggcgaagaatctcgtgctttcagcttcgatgtaggagggcgtggatatgtcctgcgggtaaatagctgcgccgatggtttctacaaagatcgttatgtttatcggcactttgcatcggccgcgctcccgattccggaagtgcttgacattggggagttcagcgagagcctgacctattgcatctcccgccgtgcacagggtgtcacgttgcaagacctgcctgaaaccgaactgcccgctgttctgcagccggtcgcggaggccatggatgcgatcgctgcggccgatcttagccagacgagcgggttcggcccattcggaccgcaaggaatcggtcaatacactacatggcgtgatttcatatgcgcgattgctgatccccatgtgtatcactggcaaactgtgatggacgacaccgtcagtgcgtccgtcgcgcaggctctcgatgagctgatgctttgggccgaggactgccccgaagtccggcacctcgtgcacgcggatttcggctccaacaatgtcctgacggacaatggccgcataacagcggtcattgactggagcgaggcgatgttcggggattcccaatacgaggtcgccaacatcttcttctggaggccgtggttggcttgtatggagcagcagacgcgctacttcgagcggaggcatccggagcttgcaggatcgccgcggctccgggcgtatatgctccgcattggtcttgaccaactctatcagagcttggttgacggcaatttcgatgatgcagcttgggcgcagggtcgatgcgacgcaatcgtccgatccggagccgggactgtcgggcgtacacaaatcgcccgcagaagcgcggccgtctggaccgatggctgtgtagaagtactcgccgatagtggaaaccgacgccccagcactcgtccgagggcaaaggaatagacgcgtgctgtaagtctgcagaaattgatgatctattaaacaataaagatgtccactaaaatggaagtttttcctgtcatactttgttaagaagggtgagaacagagtacctacattttgaatggaaggattggagctacgggggtgggggtggggtgggattagataaatgcctgctctttactgaaggctctttactattgctttatgataatgtttcatagttggatatcataatttaaacaagcaaaaccaaattaagggccagctcattcctcccactcatgatctatggatctatagatctctcgtgcagctggggctctagggggtatccccacgcgccctgtagcggcgcattaagcgcggcgggtgtggtggttacgcgcagcgtgaccgctacacttgccagcgccctagcgcccgctcctttcgctttcttcccttcctttctcgccacgttcgccggctttccccgtcaagctctaaatcgggggctccctttagggttccgatttagtgctttacggcacctcgaccccaaaaaacttgattagggtgatggttcacgtagtgggccatcgccctgatagacggtttttcgccctttgacgttggagtccacgttctttaatagtggactcttgttccaaactggaacaacactcaaccctatctcggtctattcttttgatttataagggattttgccgatttcggcctattggttaaaaaatgagctgatttaacaaaaatttaacgcgaattaattctgtggaatgtgtgtcagttagtcgcgatgtgtgactagttagttattaatagtaatcaattacggggtcattagttcatagcccatatatggagttccgcgttacataacttacggtaaatggcccgcctggctgaccgcccaacgacccccgcccattgacgtcaataatgacgtatgttcccatagtaacgccaatagggactttccattgacgtcaatgggtggagtatttacggtaaactgcccacttggcagtacatcaagtgtatcatatgccaagtacgccccctattgacgtcaatgacggtaaatggcccgcctggcattatgcccagtacatgaccttatgggactttcctacttggcagtacatctacgtattagtcatcgctattaccatggtgatgcggttttggcagtacatcaatgggcgtggatagcggtttgactcacggggatttccaagtctccaccccattgacgtcaatgggagtttgttttggcaccaaaatcaacgggactttccaaaatgtcgtaacaactccgccccattgacgcaaatgggcggtaggcgtgtacggtgggaggtctatataagcagagctcatgatagaagcactctactattcgtcgaccgatcctgagaacttcagggtgagtttggggacccttgattgttctttctttttcgctattgtaaaattcatgttatatggagggggcaaagttttcagggtgttgtttagaatgggaagatgtcccttgtatcaccatggaccctcatgataattttgtttctttcactttctactctgttgacaaccattgtctcctcttattttcttttcattttctgtaactttttcgttaaactttagcttgcatttgtaacgaatttttaaattcacttttgtttatttgtcagattgtaagtactttctctaatcacttttttttcaaggcaatcagggtatattatattgtacttcagcacagttttagagaacaattgttataattaaatgataaggtagaatatttctgcatataaattctggctggcgtggaaatattcttattggtagaaacaactacaccctggtcatcatcctgcctttctctttatggttacaatgatatacactgtttgagatgaggataaaatactctgagtccaaaccgggcccctctgctaaccatgttcatgccttcttctctttcctacagctcctgggcaacgtgctggttgttgtgctgtctcatcattttggcaaagaattaagcttatac

SEQ ID NO: 43 - protein, 115 aa, synthetic construct
  REGION 1..115: note = consensus sequence
  SITE 1: note = MISC_FEATURE - Xaa can be any naturally occurring amino acid
  SITE 11: note = MISC_FEATURE - Xaa can be any naturally occurring amino acid
  SITE 28: note = MISC_FEATURE - Xaa can be any naturally occurring amino acid
  SITE 30: note = MISC_FEATURE - Xaa can be any naturally occurring amino acid
  REGION 34..35: note = MISC_FEATURE - Xaa can be any naturally occurring amino acid
  SITE 93: note = MISC_FEATURE - Xaa can be any naturally occurring amino acid
  SITE 96: note = MISC_FEATURE - Xaa can be any naturally occurring amino acid
  SITE 100: note = MISC_FEATURE - Xaa can be any naturally occurring amino acid
  SITE 111: note = MISC_FEATURE - Xaa can be any naturally occurring amino acid
  SITE 114: note = MISC_FEATURE - Xaa can be any naturally occurring amino acid
XDVWGQGTTVXVSSASTKGPSVFPLAPXSXSTSXXTAALGCLVKDYFPEPVTVSWNSGALTSGVHTFPAVLQSSGLYSLSSVVTVPSSSLGTXTYXCNVXHKPSNTKVDKXVEXK

SEQ ID NO: 44 - protein, 225 aa, synthetic construct
  REGION 1..225: note = consensus sequence
  SITE 13: note = MISC_FEATURE - Xaa can be any naturally occurring amino acid
  SITE 47: note = MISC_FEATURE - Xaa can be any naturally occurring amino acid
  SITE 53: note = MISC_FEATURE - Xaa can be any naturally occurring amino acid
  SITE 75: note = MISC_FEATURE - Xaa can be any naturally occurring amino acid
  SITE 106: note = MISC_FEATURE - Xaa can be any naturally occurring amino acid
  REGION 109..110: note = MISC_FEATURE - Xaa can be any naturally occurring amino acid
  REGION 134..135: note = MISC_FEATURE - Xaa can be any naturally occurring amino acid
  SITE 137: note = misc_feature - Xaa can be any naturally occurring amino acid
  SITE 188: note = MISC_FEATURE - Xaa can be any naturally occurring amino acid
  SITE 198: note = MISC_FEATURE - Xaa can be any naturally occurring amino acid
  SITE 224: note = MISC_FEATURE - Xaa can be any naturally occurring amino acid
YGPPCPPCPAPEXLGGPSVFLFPPKPKDTLMISRTPEVTCVVVDVSXEDPEVXFNWYVDGVEVHNAKTKPREEQXNSTYRVVSVLTVLHQDWLNGKEYKCKVSNKXLPXXIEKTISKAKGQPREPQVYTLPPSXXEXTKNQVSLTCLVKGFYPSDIAVEWESNGQPENNYKTTPPVLDSDGSFFLYSXLTVDKSRWQXGNVFSCSVMHEALHNHYTQKSLSLSXG

SEQ ID NO: 45 - protein, 60 aa, synthetic construct
  REGION 1..60: note = consensus sequence
  REGION 13..14: note = MISC_FEATURE - Xaa can be any naturally occurring amino acid
  SITE 16: note = MISC_FEATURE - Xaa can be any naturally occurring amino acid
  REGION 21..22: note = MISC_FEATURE - Xaa can be any naturally occurring amino acid
  REGION 24..27: note = MISC_FEATURE - Xaa can be any naturally occurring amino acid
  SITE 31: note = MISC_FEATURE - Xaa can be any naturally occurring amino acid
  SITE 34: note = MISC_FEATURE - Xaa can be any naturally occurring amino acid
  SITE 48: note = MISC_FEATURE - Xaa can be any naturally occurring amino acid
  SITE 50: note = misc_feature - Xaa can be any naturally occurring amino acid
  SITE 54: note = MISC_FEATURE - Xaa can be any naturally occurring amino acid
  SITE 56: note = MISC_FEATURE - Xaa can be any naturally occurring amino acid
SDYLAWYQQKPGXXPXLLIYXXSXXXXGVPXRFXGSGSGTDFTLTISXLXPEDXAXYYCQ

SEQ ID NO: 46 - protein, 118 aa, synthetic construct
  REGION 1..118: note = consensus sequence
  SITE 4: note = MISC_FEATURE - Xaa can be any naturally occurring amino acid
TFGXGTKVEIKRTVAAPSVFIFPPSDEQLKSGTASVVCLLNNFYPREAKVQWKVDNALQSGNSQESVTEQDSKDSTYSLSSTLTLSKADYEKHKVYACEVTHQGLSSPVTKSFNRGEC